European Patent Application EP 4 722 360 A1, published April 8, 2026. Title: ＤＮＡ編集方法及びこれを用いた細胞製造方法、並びに、これらの方法に用いるためのＤＮＡ編集用ベクター及びＤＮＡ編集用キット. Applicant: Mazda Motor Corporation. The sequence listing filed with the application follows.

SEQUENCE LISTING (57 sequences)

SEQ ID NO: 1 - DNA, 504 bp, Saccharomyces cerevisiae
  source 1..504: mol_type = genomic DNA
atcacgtgctataaaaataattataatttaaattttttaatataaatatataaattaaaaatagaaagtaaaaaaagaaattaaagaaaaaatagtttttgttttccgaagatgtaaaagactctagggggatcgccaacaaatactaccttttatcttgctcttcctgctctcaggtattaatgccgaattgtttcatcttgtctgtgtagaagaccacacacgaaaatcctgtgattttacattttacttatcgttaatcgaatgtatatctatttaatctgcttttcttgtctaataaatatatatgtaaagtacgctttttgttgaaattttttaaacctttgtttatttttttttcttcattccgtaactcttctaccttctttatttactttctaaaatccaaatacaaaacataaaaataaataaacacagagtaaattcccaaattattccatcattaaaagatacgaggcgcgtgtaagttacaggcaagcgatc

SEQ ID NO: 2 - DNA, 547 bp, Nannochloropsis oceanica
  source 1..547: mol_type = genomic DNA; note = ProLHC
atgaccatgattacgccaagctatttaggtgacactataggggaaagcttgcatgcctgcaggtcgactctagaggatctactagtcatatggattggtggagtgagatagcaggagcatcacgcctcacttacggcaaccagcaacagcaacacctgcttgaagcatcaccgcgaacacaggtatgcgcttatggaccttgaacgaatccatgctgcctcaagctcccctccttgcgtgccgtcttgcttgccttaacccttctgcagacgccctagacaagaaataagaggccatccaatagatgattacagatagtggagacccaaaatgctgcacatgcgaccttatttgccattcggggctgagaatcgtgcgcagcgtcgaagccttttttctgcctccctcctctccttccttggatcacttgcttcccattcgcatgtcctgcttgctgcttccctcccccagccaccctcaagtcaaggactttacttccttcttctcacatccaacacaggtgcaactccctccttctttcccaagc

SEQ ID NO: 3 - DNA, 405 bp, synthetic construct
  source 1..405: mol_type = other DNA; note = aphVIII-5'
atggacgatgcgttgcgtgcactgcggggtcggtatcccggttgtgagtgggttgttgtggaggatggggcctcgggggctggtgtttatcggcttcggggtggtgggcgggagttgtttgtcaaggtggcagctctgggggccggggtgggcttgttgggtgaggctgagcggctggtgtggttggcggaggtggggattcccgtacctcgtgttgtggagggtggtggggacgagagggtcgcctggttggtcaccgaagcggttccggggcgtccggccagtgcgcggtggccgcgggagcagcggctggacgtggcggtggcgctcgcggggctcgctcgttcgctgcacgcgctggactgggagcggtgtccgttcgatcgcagtctcgcggtgacggtg

SEQ ID NO: 4 - DNA, 51 bp, synthetic construct
  source 1..51: mol_type = other DNA; note = T1
tctggaacatgagcccgcaaggagaggacggcggccccgccgactcgacga

SEQ ID NO: 5 - DNA, 36 bp, synthetic construct
  source 1..36: mol_type = other DNA; note = Hv1-36
ttgttccgtccgccctccgcacaaggagtctggaac

SEQ ID NO: 6 - DNA, 767 bp, Nannochloropsis oceanica
  source 1..767: mol_type = genomic DNA; note = ProLDSP
gtctctaagatggagtggatggaggaggaggcgagcgtagcagcaagcgtgagttatacagccaggcacatgtcgcaatccttcggtctcgggcttaaaatccacgcactaatcacgctgggccatgcaaagagcaatgccgaggcccaccacacaaaacgctgtgtcgcgcgttgcggcctgaagcttcatacttcttagtcgccgccaaaagggctcgagagacgagacccgttggcatgaccgatgttgttcgacgcggtttgcttcgtcacagtcgacgtgattcaggaatctggagcctgcagatcatttttttcagcctgatatcgttcttttccactgagaaccatcagaccaccttttcttccattgtgtgaaggagtaggagttgccgtgctgctttgtgggagacatctgcgatggtgaccagcctcccgtcgtctggtcgacgtgacgagcctcttcactgttcttcgacggagagacgcaagcgagacggctctagaccttttggacacgcattctgtgtgtgaactagtggacagtgataccacgtctgaaagctcaccactgcccatggtgcagctacttgtcacaaagttttgactccgtcggtatcaccattcgcgctcgtgtgcctggttgttccgccacgccggcctgccccggggcggggcaatattctaaaatctcacgcaaaacaccgcacttacccctcacacatattcgtgatagaccaccaccaatctcagcccgcatcaaca

SEQ ID NO: 7 - DNA, 36 bp, synthetic construct
  source 1..36: mol_type = other DNA; note = Hv2-36
atgagcccgcaaggagaggacggcggccccgccgac

SEQ ID NO: 8 - DNA, 607 bp, synthetic construct
  source 1..607: mol_type = other DNA; note = aphVIII-3'
gattcccgtacctcgtgttgtggagggtggtggggacgagagggtcgcctggttggtcaccgaagcggttccggggcgtccggccagtgcgcggtggccgcgggagcagcggctggacgtggcggtggcgctcgcggggctcgctcgttcgctgcacgcgctggactgggagcggtgtccgttcgatcgcagtctcgcggtgacggtgccgcaggcggcccgtgctgtcgctgaagggagcgtcgacttggaggatctggacgaggagcggaaggggtggtcgggggagcggcttctcgccgagctggagcggactcggcctgcggacgaggatctggcggtttgccacggtgacctgtgcccggacaacgtgctgctcgaccctcgtacctgcgaggtgaccgggctgatcgacgtggggcgggtcggccgtgcggaccggcactccgatctcgcgctggtgctgcgcgagctggcccacgaggaggacccgtggttcgggccggagtgttccgcggcgttcctgcgggagtacgggcgcgggtgggatggggcggtatcggaggaaaagctggcgttttaccggctgttggacgaatttttctga

SEQ ID NO: 9 - DNA, 482 bp, Nannochloropsis oceanica
  source 1..482: mol_type = genomic DNA; note = terFCP
gccgcagcctcttgggtgaagtgtttttaccccccttctccttcacccccgcattcagatgtgcagcgtaaccatacctgctatacataccttgcatcatctagaataactagaaggtcaacgacaatatcttaaaactgagattttgaacgaaagagacttaacaaacagtaggaaataggaagtaatatggaagggatacagctagtagcaaatgattgagtctaagtcctgtcgtttggttcgtgcccgcccctcgtttacatcaagaaatgaaattctcgtcagacagcaggagggagaacattcaccgttaaaagcgtgtagcctttccagagatagagatggaaaagcaagcgacctatcagccgatgaaataatttaaaaagaaaagaaagaaaaggtaacgaggattcaataattgctctgatcctacctagtcgatgataatcttgtctctccttattcttttcggttgtatt

SEQ ID NO: 10 - DNA, 18 bp, synthetic construct
  source 1..18: mol_type = other DNA; note = L1
tctggaacatgagcccgc

SEQ ID NO: 11 - DNA, 18 bp, synthetic construct
  source 1..18: mol_type = other DNA; note = R1
gccccgccgactcgacga

SEQ ID NO: 12 - DNA, 210 bp, synthetic construct
  source 1..210: mol_type = other DNA; note = Hv1-210
ccatacacgttgaacatgaacatcaggtctcttatcttcttgctcactcaccactctgctccccatacactctcttcaccaacgaaaccttgtgcaggacacggtgttgttgtcaaggtcatagcatattaaagaagaccgacggcacaaccgtccgcttaggtggtttctgcgttgttccgtccgccctccgcacaaggagtctggaac

SEQ ID NO: 13 - DNA, 210 bp, synthetic construct
  source 1..210: mol_type = other DNA; note = Hv2-210
atgagcccgcaaggagaggacggcggccccgccgactcgacgacgacgaggacgacgacgtctgaggcgatggccatgccggcaggagcagcagggacagcagccacatctgcatcagacagtcctagcagtcaccaagatgaagggggtggtcctacccaaacggtccaccgcgggccacacccggacattcacgaccagggggacaag

SEQ ID NO: 14 - DNA, 5770 bp, synthetic construct
  source 1..5770: mol_type = other DNA; note = pNICS36
tttcctgcgttatcccctgattctgtggataaccgtattaccgcctttgagtgagctgataccgctcgccgcagccgaacgaccgagcgcagcgagtcagtgagcgaggaagcggaagagcgcccaatacgcaaaccgcctctccccgcgcgttggccgattcattaatgcagctgcggccgccggttgtattaatcgggatcccctcgaattcacgatgcggtattttctccttacgcatctgtgcggtatttcacaccaagtgccacctgggtccttttcatcacgtgctataaaaataattataatttaaattttttaatataaatatataaattaaaaatagaaagtaaaaaaagaaattaaagaaaaaatagtttttgttttccgaagatgtaaaagactctagggggatcgccaacaaatactaccttttatcttgctcttcctgctctcaggtattaatgccgaattgtttcatcttgtctgtgtagaagaccacacacgaaaatcctgtgattttacattttacttatcgttaatcgaatgtatatctatttaatctgcttttcttgtctaataaatatatatgtaaagtacgctttttgttgaaattttttaaacctttgtttatttttttttcttcattccgtaactcttctaccttctttatttactttctaaaatccaaatacaaaacataaaaataaataaacacagagtaaattcccaaattattccatcattaaaagatacgaggcgcgtgtaagttacaggcaagcgatcccaaaaggccaggaaccgtaaaaaggccgcgttgctggcgtttttccataggctccgcccccctgacgagcatcacaaaaatcgacgctcaagtcagaggtggcgaaacccgacaggactataaagataccaggcgtttccccctggaagctccctcgtgcgctctcctgttccgaccctgccgcttaccggatacctgtccgcctttctcccttcgggaagcgtggcgctttctcatagctcacgctgtaggtatctcagttcggtgtaggtcgttcgctccaagctgggctgtgtgcacgaaccccccgttcagcccgaccgctgcgccttatccggtaactatcgtcttgagtccaacccggtaagacacgacttatcgccactggcagcagccactggtaacaggattagcagagcgaggtatgtaggcggtgctacagagttcttgaagtggtggcctaactacggctacactagaagaacagtatttggtatctgcgctctgctgaagccagttaccttcggaaaaagagttggtagctcttgatccggcaaacaaaccaccgctggtagcggtggtttttttgtttgcaagcagcagattacgcgcagaaaaaaaggatctcaagaagatcctttgatcttttctacggggtctgacgctcagtggaacgaaaactcacgttaagggattttggtcatgagattatcaaaaaggatcttcacctagatccttttaaattaaaaatgaagttttaaatcaatctaaagtatatatgagtaaacttggtctgacagttaccaatgcttaatcagtgaggcacctatctcagcgatctgtctatttcgttcatccatagttgcctgactccccgtcgtgtagataactacgatacgggagggcttaccatctggccccagtgctgcaatgataccgcgagacccacgctcaccggctccagatttatcagcaataaaccagccagccggaagggccgagcgcagaagtggtcctgcaactttatccgcctccatccagtctattaattgttgccgggaagctagagtaagtagttcgccagttaatagtttgcgcaacgttgttgccattgctacaggcatcgtggtgtcacgctcgtcgtttggtatggcttcattcagctccggttcccaacgatcaaggcgagttacatgatcccccatgttgtgcaaaaaagcggttagctccttcggtcctccgatcgttgtcagaagtaagttggccgcagtgttatcactcatggttatggcagcactgcataattctcttactgtcatgccatccgtaagatgcttttctgtgactggtgagtactcaaccaagtcattctgagaatagtgtatgcggcgaccgagttgctcttgcccggcgtcaatacgggataataccgcgccacatagcagaactttaaaagtgctcatcattggaaaacgttcttcggggcgaaaactctcaaggatcttaccgctgttgagatccagttcgatgtaacccactcgtgcacccaactgatcttcagcatcttttactttcaccagcgtttctgggtgagcaaaaacaggaaggcaaaatgccgcaaaaaagggaataagggcgacacggaaatgttgaatactcatactcttcctttttcaatattattgaagcatttatcagggttattgtctcatgagcggatacatatttgaatgtatttagaaaaataaacaaataggggttccgcgcacatttccccgaaaagtgccacctgacgtctaagaaaccattattatcatgacattaacctataaaaataggcgtatcacgaggccctttcgtctggcgcgtttcggtgatgacggtgaaaacctctgacacatgcagctcccgatatcggtcacagcttgtctgtaagcggatgccgggagcagacaagcccgtcagggcgcgtcagcgggtgttggcgggtgtcgggatgaccatgattacgccaagctatttaggtgacactataggggaaagcttgcatgcctgcaggtcgactctagaggatctactagtcatatggattggtggagtgagatagcaggagcatcacgcctcacttacggcaaccagcaacagcaacacctgcttgaagcatcaccgcgaacacaggtatgcgcttatggaccttgaacgaatccatgctgcctcaagctcccctccttgcgtgccgtcttgcttgccttaacccttctgcagacgccctagacaagaaataagaggccatccaatagatgattacagatagtggagacccaaaatgctgcacatgcgaccttatttgccattcggggctgagaatcgtgcgcagcgtcgaagccttttttctgcctccctcctctccttccttggatcacttgcttcccattcgcatgtcctgcttgctgcttccctcccccagccaccctcaagtcaaggactttacttccttcttctcacatccaacacaggtgcaactccctccttctttcccaagcatggacgatgcgttgcgtgcactgcggggtcggtatcccggttgtgagtgggttgttgtggaggatggggcctcgggggctggtgtttatcggcttcggggtggtgggcgggagttgtttgtcaaggtggcagctctgggggccggggtgggcttgttgggtgaggctgagcggctggtgtggttggcggaggtggggattcccgtacctcgtgttgtggagggtggtggggacgagagggtcgcctggttggtcaccgaagcggttccggggcgtccggccagtgcgcggtggccgcgggagcagcggctggacgtggcggtggcgctcgcggggctcgctcgttcgctgcacgcgctggactgggagcggtgtccgttcgatcgcagtctcgcggtgacggtgtagtctggaacatgagcccgcaaggagaggacggcggccccgccgactcgacgattgttccgtccgccctccgcacaaggagtctggaacgtctctaagatggagtggatggaggaggaggcgagcgtagcagcaagcgtgagttatacagccaggcacatgtcgcaatccttcggtctcgggcttaaaatccacgcactaatcacgctgggccatgcaaagagcaatgccgaggcccaccacacaaaacgctgtgtcgcgcgttgcggcctgaagcttcatacttcttagtcgccgccaaaagggctcgagagacgagacccgttggcatgaccgatgttgttcgacgcggtttgcttcgtcacagtcgacgtgattcaggaatctggagcctgcagatcatttttttcagcctgatatcgttcttttccactgagaaccatcagaccaccttttcttccattgtgtgaaggagtaggagttgccgtgctgctttgtgggagacatctgcgatggtgaccagcctcccgtcgtctggtcgacgtgacgagcctcttcactgttcttcgacggagagacgcaagcgagacggctctagaccttttggacacgcattctgtgtgtgaactagtggacagtgataccacgtctgaaagctcaccactgcccatggtgcagctacttgtcacaaagttttgactccgtcggtatcaccattcgcgctcgtgtgcctggttgttccgccacgccggcctgccccggggcggggcaatattctaaaatctcacgcaaaacaccgcacttacccctcacacatattcgtgatagaccaccaccaatctcagcccgcatcaacaatgagcccgcaaggagaggacggcggccccgccgactctggaacatgagcccgcaaggagaggacggcggccccgccgactcgacgatagattcccgtacctcgtgttgtggagggtggtggggacgagagggtcgcctggttggtcaccgaagcggttccggggcgtccggccagtgcgcggtggccgcgggagcagcggctggacgtggcggtggcgctcgcggggctcgctcgttcgctgcacgcgctggactgggagcggtgtccgttcgatcgcagtctcgcggtgacggtgccgcaggcggcccgtgctgtcgctgaagggagcgtcgacttggaggatctggacgaggagcggaaggggtggtcgggggagcggcttctcgccgagctggagcggactcggcctgcggacgaggatctggcggtttgccacggtgacctgtgcccggacaacgtgctgctcgaccctcgtacctgcgaggtgaccgggctgatcgacgtggggcgggtcggccgtgcggaccggcactccgatctcgcgctggtgctgcgcgagctggcccacgaggaggacccgtggttcgggccggagtgttccgcggcgttcctgcgggagtacgggcgcgggtgggatggggcggtatcggaggaaaagctggcgttttaccggctgttggacgaatttttctgagccgcagcctcttgggtgaagtgtttttaccccccttctccttcacccccgcattcagatgtgcagcgtaaccatacctgctatacataccttgcatcatctagaataactagaaggtcaacgacaatatcttaaaactgagattttgaacgaaagagacttaacaaacagtaggaaataggaagtaatatggaagggatacagctagtagcaaatgattgagtctaagtcctgtcgtttggttcgtgcccgcccctcgtttacatcaagaaatgaaattctcgtcagacagcaggagggagaacattcaccgttaaaagcgtgtagcctttccagagatagagatggaaaagcaagcgacctatcagccgatgaaataatttaaaaagaaaagaaagaaaaggtaacgaggattcaataattgctctgatcctacctagtcgatgataatcttgtctctccttattcttttcggttgtatt

SEQ ID NO: 15 - DNA, 6118 bp, synthetic construct
  source 1..6118: mol_type = other DNA; note = pNICS210
tttcctgcgttatcccctgattctgtggataaccgtattaccgcctttgagtgagctgataccgctcgccgcagccgaacgaccgagcgcagcgagtcagtgagcgaggaagcggaagagcgcccaatacgcaaaccgcctctccccgcgcgttggccgattcattaatgcagctgcggccgccggttgtattaatcgggatcccctcgaattcacgatgcggtattttctccttacgcatctgtgcggtatttcacaccaagtgccacctgggtccttttcatcacgtgctataaaaataattataatttaaattttttaatataaatatataaattaaaaatagaaagtaaaaaaagaaattaaagaaaaaatagtttttgttttccgaagatgtaaaagactctagggggatcgccaacaaatactaccttttatcttgctcttcctgctctcaggtattaatgccgaattgtttcatcttgtctgtgtagaagaccacacacgaaaatcctgtgattttacattttacttatcgttaatcgaatgtatatctatttaatctgcttttcttgtctaataaatatatatgtaaagtacgctttttgttgaaattttttaaacctttgtttatttttttttcttcattccgtaactcttctaccttctttatttactttctaaaatccaaatacaaaacataaaaataaataaacacagagtaaattcccaaattattccatcattaaaagatacgaggcgcgtgtaagttacaggcaagcgatcccaaaaggccaggaaccgtaaaaaggccgcgttgctggcgtttttccataggctccgcccccctgacgagcatcacaaaaatcgacgctcaagtcagaggtggcgaaacccgacaggactataaagataccaggcgtttccccctggaagctccctcgtgcgctctcctgttccgaccctgccgcttaccggatacctgtccgcctttctcccttcgggaagcgtggcgctttctcatagctcacgctgtaggtatctcagttcggtgtaggtcgttcgctccaagctgggctgtgtgcacgaaccccccgttcagcccgaccgctgcgccttatccggtaactatcgtcttgagtccaacccggtaagacacgacttatcgccactggcagcagccactggtaacaggattagcagagcgaggtatgtaggcggtgctacagagttcttgaagtggtggcctaactacggctacactagaagaacagtatttggtatctgcgctctgctgaagccagttaccttcggaaaaagagttggtagctcttgatccggcaaacaaaccaccgctggtagcggtggtttttttgtttgcaagcagcagattacgcgcagaaaaaaaggatctcaagaagatcctttgatcttttctacggggtctgacgctcagtggaacgaaaactcacgttaagggattttggtcatgagattatcaaaaaggatcttcacctagatccttttaaattaaaaatgaagttttaaatcaatctaaagtatatatgagtaaacttggtctgacagttaccaatgcttaatcagtgaggcacctatctcagcgatctgtctatttcgttcatccatagttgcctgactccccgtcgtgtagataactacgatacgggagggcttaccatctggccccagtgctgcaatgataccgcgagacccacgctcaccggctccagatttatcagcaataaaccagccagccggaagggccgagcgcagaagtggtcctgcaactttatccgcctccatccagtctattaattgttgccgggaagctagagtaagtagttcgccagttaatagtttgcgcaacgttgttgccattgctacaggcatcgtggtgtcacgctcgtcgtttggtatggcttcattcagctccggttcccaacgatcaaggcgagttacatgatcccccatgttgtgcaaaaaagcggttagctccttcggtcctccgatcgttgtcagaagtaagttggccgcagtgttatcactcatggttatggcagcactgcataattctcttactgtcatgccatccgtaagatgcttttctgtgactggtgagtactcaaccaagtcattctgagaatagtgtatgcggcgaccgagttgctcttgcccggcgtcaatacgggataataccgcgccacatagcagaactttaaaagtgctcatcattggaaaacgttcttcggggcgaaaactctcaaggatcttaccgctgttgagatccagttcgatgtaacccactcgtgcacccaactgatcttcagcatcttttactttcaccagcgtttctgggtgagcaaaaacaggaaggcaaaatgccgcaaaaaagggaataagggcgacacggaaatgttgaatactcatactcttcctttttcaatattattgaagcatttatcagggttattgtctcatgagcggatacatatttgaatgtatttagaaaaataaacaaataggggttccgcgcacatttccccgaaaagtgccacctgacgtctaagaaaccattattatcatgacattaacctataaaaataggcgtatcacgaggccctttcgtctggcgcgtttcggtgatgacggtgaaaacctctgacacatgcagctcccgatatcggtcacagcttgtctgtaagcggatgccgggagcagacaagcccgtcagggcgcgtcagcgggtgttggcgggtgtcgggatgaccatgattacgccaagctatttaggtgacactataggggaaagcttgcatgcctgcaggtcgactctagaggatctactagtcatatggattggtggagtgagatagcaggagcatcacgcctcacttacggcaaccagcaacagcaacacctgcttgaagcatcaccgcgaacacaggtatgcgcttatggaccttgaacgaatccatgctgcctcaagctcccctccttgcgtgccgtcttgcttgccttaacccttctgcagacgccctagacaagaaataagaggccatccaatagatgattacagatagtggagacccaaaatgctgcacatgcgaccttatttgccattcggggctgagaatcgtgcgcagcgtcgaagccttttttctgcctccctcctctccttccttggatcacttgcttcccattcgcatgtcctgcttgctgcttccctcccccagccaccctcaagtcaaggactttacttccttcttctcacatccaacacaggtgcaactccctccttctttcccaagcatggacgatgcgttgcgtgcactgcggggtcggtatcccggttgtgagtgggttgttgtggaggatggggcctcgggggctggtgtttatcggcttcggggtggtgggcgggagttgtttgtcaaggtggcagctctgggggccggggtgggcttgttgggtgaggctgagcggctggtgtggttggcggaggtggggattcccgtacctcgtgttgtggagggtggtggggacgagagggtcgcctggttggtcaccgaagcggttccggggcgtccggccagtgcgcggtggccgcgggagcagcggctggacgtggcggtggcgctcgcggggctcgctcgttcgctgcacgcgctggactgggagcggtgtccgttcgatcgcagtctcgcggtgacggtgtagtctggaacatgagcccgcaaggagaggacggcggccccgccgactcgacgaccatacacgttgaacatgaacatcaggtctcttatcttcttgctcactcaccactctgctccccatacactctcttcaccaacgaaaccttgtgcaggacacggtgttgttgtcaaggtcatagcatattaaagaagaccgacggcacaaccgtccgcttaggtggtttctgcgttgttccgtccgccctccgcacaaggagtctggaacgtctctaagatggagtggatggaggaggaggcgagcgtagcagcaagcgtgagttatacagccaggcacatgtcgcaatccttcggtctcgggcttaaaatccacgcactaatcacgctgggccatgcaaagagcaatgccgaggcccaccacacaaaacgctgtgtcgcgcgttgcggcctgaagcttcatacttcttagtcgccgccaaaagggctcgagagacgagacccgttggcatgaccgatgttgttcgacgcggtttgcttcgtcacagtcgacgtgattcaggaatctggagcctgcagatcatttttttcagcctgatatcgttcttttccactgagaaccatcagaccaccttttcttccattgtgtgaaggagtaggagttgccgtgctgctttgtgggagacatctgcgatggtgaccagcctcccgtcgtctggtcgacgtgacgagcctcttcactgttcttcgacggagagacgcaagcgagacggctctagaccttttggacacgcattctgtgtgtgaactagtggacagtgataccacgtctgaaagctcaccactgcccatggtgcagctacttgtcacaaagttttgactccgtcggtatcaccattcgcgctcgtgtgcctggttgttccgccacgccggcctgccccggggcggggcaatattctaaaatctcacgcaaaacaccgcacttacccctcacacatattcgtgatagaccaccaccaatctcagcccgcatcaacaatgagcccgcaaggagaggacggcggccccgccgactcgacgacgacgaggacgacgacgtctgaggcgatggccatgccggcaggagcagcagggacagcagccacatctgcatcagacagtcctagcagtcaccaagatgaagggggtggtcctacccaaacggtccaccgcgggccacacccggacattcacgaccagggggacaagtctggaacatgagcccgcaaggagaggacggcggccccgccgactcgacgatagattcccgtacctcgtgttgtggagggtggtggggacgagagggtcgcctggttggtcaccgaagcggttccggggcgtccggccagtgcgcggtggccgcgggagcagcggctggacgtggcggtggcgctcgcggggctcgctcgttcgctgcacgcgctggactgggagcggtgtccgttcgatcgcagtctcgcggtgacggtgccgcaggcggcccgtgctgtcgctgaagggagcgtcgacttggaggatctggacgaggagcggaaggggtggtcgggggagcggcttctcgccgagctggagcggactcggcctgcggacgaggatctggcggtttgccacggtgacctgtgcccggacaacgtgctgctcgaccctcgtacctgcgaggtgaccgggctgatcgacgtggggcgggtcggccgtgcggaccggcactccgatctcgcgctggtgctgcgcgagctggcccacgaggaggacccgtggttcgggccggagtgttccgcggcgttcctgcgggagtacgggcgcgggtgggatggggcggtatcggaggaaaagctggcgttttaccggctgttggacgaatttttctgagccgcagcctcttgggtgaagtgtttttaccccccttctccttcacccccgcattcagatgtgcagcgtaaccatacctgctatacataccttgcatcatctagaataactagaaggtcaacgacaatatcttaaaactgagattttgaacgaaagagacttaacaaacagtaggaaataggaagtaatatggaagggatacagctagtagcaaatgattgagtctaagtcctgtcgtttggttcgtgcccgcccctcgtttacatcaagaaatgaaattctcgtcagacagcaggagggagaacattcaccgttaaaagcgtgtagcctttccagagatagagatggaaaagcaagcgacctatcagccgatgaaataatttaaaaagaaaagaaagaaaaggtaacgaggattcaataattgctctgatcctacctagtcgatgataatcttgtctctccttattcttttcggttgtatt

SEQ ID NO: 16 - DNA, 2997 bp, synthetic construct
  source 1..2997: mol_type = other DNA; note = TALEN-L
atggcctcctccccccccaagaaaaagcgcaaggtcgccgccgccgattacaaggacgacgacgacaagtcctggaaagacgcgtccggttggtcccgaatgcatgccgcccctcgccgccgcgcggcccagccctccgacgcctcccccgccgcccaagtcgacctccgaaccttgggttactctcagcagcagcaggagaagatcaagcctaaggtccgctccaccgtcgcgcagcatcacgaggccctcgtcggccacggtttcacccatgcccacattgtggccctctcccagcatcccgccgccttgggcacggtggccgtgacgtaccagcacatcatcacggccctccccgaggccacccacgaggatatcgtgggtgtcggtaaacagtggtccggcgcccgcgccttggaggccctcctcaccgatgccggcgaactccgaggtcctcctctccaactcgacaccggccagttggtcaagattgccaagcgcggcggtgtcaccgccatggaggccgtccatgcgtcccgcaacgccttgaccggcgcccccctcaacctgaccccggaccaggtggttgcaatcgcgtcacacgatgggggaaagcaggccctagaaaccgttcagcgactcctgcccgtcctgtgccaggaccacggcctgacccccgaacaggttgtcgctattgctagtaacggcggaggcaaacaggcgctggaaacagttcagcgcctcttgccggtcttgtgtcaggcccacggcctgaccccagaccaagttgtcgcgattgcaagcaacaacggaggcaaacaagccttagaaacagtccagagattgttgcctgtgctgtgccaagcccacggcctgaccccagcccaagttgtcgcgattgcaagcaacaacggaggcaaacaagccttagaaacagtccagagattgttgccggtgctgtgccaagaccacggcctgaccccagaccaggttgtggccatcgccagcaacataggtggcaagcaggccctcgaaaccgtccagagactgttaccggttctctgccaggaccacggcctgaccccagaacaggttgtggccatcgccagcaacataggtggcaagcaggccctcgaaaccgtccagagactgttaccggttctctgccaggcccacggcctgaccccggaccaggtggttgcaatcgcgtcacacgatgggggaaagcaggccctagaaaccgttcagcgactcctgcccgtcctgtgccaggcccacggcctgaccccagcccaggttgtggccatcgccagcaacataggtggcaagcaggccctcgaaaccgtccagagactgttaccggttctctgccaggaccacggcctgacccccgaccaggttgtcgctattgctagtaacggcggaggcaaacaggcgctggaaacagttcagcgcctcttgccggtcttgtgtcaggaccacggcctgaccccagaacaagttgtcgcgattgcaagcaacaacggaggcaaacaagccttagaaacagtccagagattgttgccggtgctgtgccaagcccacggcctgaccccagaccaggttgtggccatcgccagcaacataggtggcaagcaggccctcgaaaccgtccagagactgttaccggttctctgccaggcccacggcctgaccccagcccaagttgtcgcgattgcaagcaacaacggaggcaaacaagccttagaaacagtccagagattgttgccggtgctgtgccaagaccacggcctgaccccggaccaggtggttgcaatcgcgtcacacgatgggggaaagcaggccctagaaaccgttcagcgactcctgcccgtcctgtgccaggaccacggcctgaccccggaacaggtggttgcaatcgcgtcacacgatgggggaaagcaggccctagaaaccgttcagcgactcctgcccgtcctgtgccaggcccacggcctgaccccggaccaggtggttgcaatcgcgtcacacgatgggggaaagcaggccctagaaaccgttcagcgactcctgcccgtcctgtgccaggcccacggcctgaccccagcccaagttgtcgcgattgcaagcaacaacggaggcaaacaagccttagaaacagtccagagattgttgccggtgctgtgccaagaccacggcctgacccccgaacaggtcgtcgccatcgcctctaacggtggtggccgacccgccctcgaatccatcgtggcgcagctctctcgacccgatcccgccttggccgccctcacgaatgaccacctcgtcgccctcgcctgtttgggcggtcgacccgccatggacgcggtcaagaagggcctccctcacgcccctgagctcatccgctcccagctcgtcaagtccgaactcgaggagaagaagtccgagctccgacacaagttgaagtacgtcccccacgagtacatcgagttgatcgagattgcccgcaactccacccaggaccgcatcctcgagatgaaggtcatggagttttttatgaaagtctacggttaccgcggtaagcacctcggtggttcccgcaagcccgatggtgccatctatacggtgggttctcccatcgactacggtgtcatcgtggacaccaaggcgtactccggtggctacaacctccccatcggccaggccgacgagatgcaacgatatgtggaggagaaccagacccgcaacaagcacatcaaccccaacgagtggtggaaggtctacccttcctccgtcaccgagttcaagttcttgtttgtttctggtcatttcaagggtaactacaaggcccaactcacccgactcaaccacatcaccaactgcaacggcgccgtcctctccgtcgaggagctcttgatcggcggcgaaatgatcaaggccggtaccctcaccctcgaggaggtccgccgcaagtttaacaacggcgagatcaacttttga

SEQ ID NO: 17 - DNA, 2997 bp, synthetic construct
  source 1..2997: mol_type = other DNA; note = TALEN-R
atggcctcctccccccccaagaaaaagcgcaaggtcgccgccgccgattacaaggacgacgacgacaagtcctggaaagacgcgtccggttggtcccgaatgcatgccgcccctcgccgccgcgcggcccagccctccgacgcctcccccgccgcccaagtcgacctccgaaccttgggttactctcagcagcagcaggagaagatcaagcctaaggtccgctccaccgtcgcgcagcatcacgaggccctcgtcggccacggtttcacccatgcccacattgtggccctctcccagcatcccgccgccttgggcacggtggccgtgacgtaccagcacatcatcacggccctccccgaggccacccacgaggatatcgtgggtgtcggtaaacagtggtccggcgcccgcgccttggaggccctcctcaccgatgccggcgaactccgaggtcctcctctccaactcgacaccggccagttggtcaagattgccaagcgcggcggtgtcaccgccatggaggccgtccatgcgtcccgcaacgccttgaccggcgcccccctcaacctgaccccggaccaggtggttgcaatcgcgtcacacgatgggggaaagcaggccctagaaaccgttcagcgactcctgcccgtcctgtgccaggaccacggcctgaccccagaacaagttgtcgcgattgcaagcaacaacggaggcaaacaagccttagaaacagtccagagattgttgccggtgctgtgccaagcccacggcctgacccccgaccaggttgtcgctattgctagtaacggcggaggcaaacaggcgctggaaacagttcagcgcctcttgccggtcttgtgtcaggcccacggcctgaccccggcccaggtggttgcaatcgcgtcacacgatgggggaaagcaggccctagaaaccgttcagcgactcctgcccgtcctgtgccaggaccacggcctgaccccagaccaagttgtcgcgattgcaagcaacaacggaggcaaacaagccttagaaacagtccagagattgttgccggtgctgtgccaagaccacggcctgaccccagaacaggttgtggccatcgccagcaacataggtggcaagcaggccctcgaaaccgtccagagactgttaccggttctctgccaggcccacggcctgaccccggaccaggtggttgcaatcgcgtcacacgatgggggaaagcaggccctagaaaccgttcagcgactcctgcccgtcctgtgccaggcccacggcctgacccccgcccaggttgtcgctattgctagtaacggcggaggcaaacaggcgctggaaacagttcagcgcctcttgccggtcttgtgtcaggaccacggcctgaccccggaccaggtggttgcaatcgcgtcacacgatgggggaaagcaggccctagaaaccgttcagcgactcctgcccgtcctgtgccaggaccacggcctgaccccagaacaagttgtcgcgattgcaagcaacaacggaggcaaacaagccttagaaacagtccagagattgttgccggtgctgtgccaagcccacggcctgaccccagaccaagttgtcgcgattgcaagcaacaacggaggcaaacaagccttagaaacagtccagagattgttgcctgtgctgtgccaagcccacggcctgaccccggcccaggtggttgcaatcgcgtcacacgatgggggaaagcaggccctagaaaccgttcagcgactcctgcccgtcctgtgccaggaccacggcctgaccccagaccaagttgtcgcgattgcaagcaacaacggaggcaaacaagccttagaaacagtccagagattgttgccggtgctgtgccaagaccacggcctgaccccagaacaagttgtcgcgattgcaagcaacaacggaggcaaacaagccttagaaacagtccagagattgttgccggtgctgtgccaagcccacggcctgaccccagaccaagttgtcgcgattgcaagcaacaacggaggcaaacaagccttagaaacagtccagagattgttgcctgtgctgtgccaagcccacggcctgaccccagcccaagttgtcgcgattgcaagcaacaacggaggcaaacaagccttagaaacagtccagagattgttgccggtgctgtgccaagaccacggcctgacccccgaacaggtcgtcgccatcgcctctaacggtggtggccgacccgccctcgaatccatcgtggcgcagctctctcgacccgatcccgccttggccgccctcacgaatgaccacctcgtcgccctcgcctgtttgggcggtcgacccgccatggacgcggtcaagaagggcctccctcacgcccctgagctcatccgctcccagctcgtcaagtccgaactcgaggagaagaagtccgagctccgacacaagttgaagtacgtcccccacgagtacatcgagttgatcgagattgcccgcaactccacccaggaccgcatcctcgagatgaaggtcatggagttttttatgaaagtctacggttaccgcggtaagcacctcggtggttcccgcaagcccgatggtgccatctatacggtgggttctcccatcgactacggtgtcatcgtggacaccaaggcgtactccggtggctacaacctccccatcggccaggccgacgagatgcaacgatatgtggaggagaaccagacccgcaacaagcacatcaaccccaacgagtggtggaaggtctacccttcctccgtcaccgagttcaagttcttgtttgtttctggtcatttcaagggtaactacaaggcccaactcacccgactcaaccacatcaccaactgcaacggcgccgtcctctccgtcgaggagctcttgatcggcggcgaaatgatcaaggccggtaccctcaccctcgaggaggtccgccgcaagtttaacaacggcgagatcaacttttga

SEQ ID NO: 18 - DNA, 14785 bp, synthetic construct
  source 1..14785: mol_type = other DNA; note = all-in-one NICS36
ttcctgcgttatcccctgattctgtggataaccgtattaccgcctttgagtgagctgataccgctcgccgcagccgaacgaccgagcgcagcgagtcagtgagcgaggaagcggaagagcgcccaatacgcaaaccgcctctccccgcgcgttggccgattcattaatgcagctgcggccgcatgaccatgattacgccaagctatttaggtgacactataggggaaagcttgcatgcctgcaggtcgactctagaggatctactagtcatatggattggtggagtgagatagcaggagcatcacgcctcacttacggcaaccagcaacagcaacacctgcttgaagcatcaccgcgaacacaggtatgcgcttatggaccttgaacgaatccatgctgcctcaagctcccctccttgcgtgccgtcttgcttgccttaacccttctgcagacgccctagacaagaaataagaggccatccaatagatgattacagatagtggagacccaaaatgctgcacatgcgaccttatttgccattcggggctgagaatcgtgcgcagcgtcgaagccttttttctgcctccctcctctccttccttggatcacttgcttcccattcgcatgtcctgcttgctgcttccctcccccagccaccctcaagtcaaggactttacttccttcttctcacatccaacacaggtgcaactccctccttctttcccaagcatggcctcctccccccccaagaaaaagcgcaaggtcgccgccgccgattacaaggacgacgacgacaagtcctggaaagacgcgtccggttggtcccgaatgcatgccgcccctcgccgccgcgcggcccagccctccgacgcctcccccgccgcccaagtcgacctccgaaccttgggttactctcagcagcagcaggagaagatcaagcctaaggtccgctccaccgtcgcgcagcatcacgaggccctcgtcggccacggtttcacccatgcccacattgtggccctctcccagcatcccgccgccttgggcacggtggccgtgacgtaccagcacatcatcacggccctccccgaggccacccacgaggatatcgtgggtgtcggtaaacagtggtccggcgcccgcgccttggaggccctcctcaccgatgccggcgaactccgaggtcctcctctccaactcgacaccggccagttggtcaagattgccaagcgcggcggtgtcaccgccatggaggccgtccatgcgtcccgcaacgccttgaccggcgcccccctcaacctgaccccggaccaggtggttgcaatcgcgtcacacgatgggggaaagcaggccctagaaaccgttcagcgactcctgcccgtcctgtgccaggaccacggcctgacccccgaacaggttgtcgctattgctagtaacggcggaggcaaacaggcgctggaaacagttcagcgcctcttgccggtcttgtgtcaggcccacggcctgaccccagaccaagttgtcgcgattgcaagcaacaacggaggcaaacaagccttagaaacagtccagagattgttgcctgtgctgtgccaagcccacggcctgaccccagcccaagttgtcgcgattgcaagcaacaacggaggcaaacaagccttagaaacagtccagagattgttgccggtgctgtgccaagaccacggcctgaccccagaccaggttgtggccatcgccagcaacataggtggcaagcaggccctcgaaaccgtccagagactgttaccggttctctgccaggaccacggcctgaccccagaacaggttgtggccatcgccagcaacataggtggcaagcaggccctcgaaaccgtccagagactgttaccggttctctgccaggcccacggcctgaccccggaccaggtggttgcaatcgcgtcacacgatgggggaaagcaggccctagaaaccgttcagcgactcctgcccgtcctgtgccaggcccacggcctgaccccagcccaggttgtggccatcgccagcaacataggtggcaagcaggccctcgaaaccgtccagagactgttaccggttctctgccaggaccacggcctgacccccgaccaggttgtcgctattgctagtaacggcggaggcaaacaggcgctggaaacagttcagcgcctcttgccggtcttgtgtcaggaccacggcctgaccccagaacaagttgtcgcgattgcaagcaacaacggaggcaaacaagccttagaaacagtccagagattgttgccggtgctgtgccaagcccacggcctgaccccagaccaggttgtggccatcgccagcaacataggtggcaagcaggccctcgaaaccgtccagagactgttaccggttctctgccaggcccacggcctgaccccagcccaagttgtcgcgattgcaagcaacaacggaggcaaacaagccttagaaacagtccagagattgttgccggtgctgtgccaagaccacggcctgaccccggaccaggtggttgcaatcgcgtcacacgatgggggaaagcaggccctagaaaccgttcagcgactcctgcccgtcctgtgccaggaccacggcctgaccccggaacaggtggttgcaatcgcgtcacacgatgggggaaagcaggccctagaaaccgttcagcgactcctgcccgtcctgtgccaggcccacggcctgaccccggaccaggtggttgcaatcgcgtcacacgatgggggaaagcaggccctagaaaccgttcagcgactcctgcccgtcctgtgccaggcccacggcctgaccccagcccaagttgtcgcgattgcaagcaacaacggaggcaaacaagccttagaaacagtccagagattgttgccggtgctgtgccaagaccacggcctgacccccgaacaggtcgtcgccatcgcctctaacggtggtggccgacccgccctcgaatccatcgtggcgcagctctctcgacccgatcccgccttggccgccctcacgaatgaccacctcgtcgccctcgcctgtttgggcggtcgacccgccatggacgcggtcaagaagggcctccctcacgcccctgagctcatccgctcccagctcgtcaagtccgaactcgaggagaagaagtccgagctccgacacaagttgaagtacgtcccccacgagtacatcgagttgatcgagattgcccgcaactccacccaggaccgcatcctcgagatgaaggtcatggagttttttatgaaagtctacggttaccgcggtaagcacctcggtggttcccgcaagcccgatggtgccatctatacggtgggttctcccatcgactacggtgtcatcgtggacaccaaggcgtactccggtggctacaacctccccatcggccaggccgacgagatgcaacgatatgtggaggagaaccagacccgcaacaagcacatcaaccccaacgagtggtggaaggtctacccttcctccgtcaccgagttcaagttcttgtttgtttctggtcatttcaagggtaactacaaggcccaactcacccgactcaaccacatcaccaactgcaacggcgccgtcctctccgtcgaggagctcttgatcggcggcgaaatgatcaaggccggtaccctcaccctcgaggaggtccgccgcaagtttaacaacggcgagatcaacttttgagccgcagcctcttgggtgaagtgtttttaccccccttctccttcacccccgcattcagatgtgcagcgtaaccatacctgctatacataccttgcatcatctagaataactagaaggtcaacgacaatatcttaaaactgagattttgaacgaaagagacttaacaaacagtaggaaataggaagtaatatggaagggatacagctagtagcaaatgattgagtctaagtcctgtcgtttggttcgtgcccgcccctcgtttacatcaagaaatgaaattctcgtcagacagcaggagggagaacattcaccgttaaaagcgtgtagcctttccagagatagagatggaaaagcaagcgacctatcagccgatgaaataatttaaaaagaaaagaaagaaaaggtaacgaggattcaataattgctctgatcctacctagtcgatgataatcttgtctctccttattcttttcggttgtattaatcgggatccatgaccatgattacgccaagctatttaggtgacactataggggaaagcttgcatgcctgcaggtcgactctagaggatctactagtcatatggattggtggagtgagatagcaggagcatcacgcctcacttacggcaaccagcaacagcaacacctgcttgaagcatcaccgcgaacacaggtatgcgcttatggaccttgaacgaatccatgctgcctcaagctcccctccttgcgtgccgtcttgcttgccttaacccttctgcagacgccctagacaagaaataagaggccatccaatagatgattacagatagtggagacccaaaatgctgcacatgcgaccttatttgccattcggggctgagaatcgtgcgcagcgtcgaagccttttttctgcctccctcctctccttccttggatcacttgcttcccattcgcatgtcctgcttgctgcttccctcccccagccaccctcaagtcaaggactttacttccttcttctcacatccaacacaggtgcaactccctccttctttcccaagcatggcctcctccccccccaagaaaaagcgcaaggtcgccgccgccgattacaaggacgacgacgacaagtcctggaaagacgcgtccggttggtcccgaatgcatgccgcccctcgccgccgcgcggcccagccctccgacgcctcccccgccgcccaagtcgacctccgaaccttgggttactctcagcagcagcaggagaagatcaagcctaaggtccgctccaccgtcgcgcagcatcacgaggccctcgtcggccacggtttcacccatgcccacattgtggccctctcccagcatcccgccgccttgggcacggtggccgtgacgtaccagcacatcatcacggccctccccgaggccacccacgaggatatcgtgggtgtcggtaaacagtggtccggcgcccgcgccttggaggccctcctcaccgatgccggcgaactccgaggtcctcctctccaactcgacaccggccagttggtcaagattgccaagcgcggcggtgtcaccgccatggaggccgtccatgcgtcccgcaacgccttgaccggcgcccccctcaacctgaccccggaccaggtggttgcaatcgcgtcacacgatgggggaaagcaggccctagaaaccgttcagcgactcctgcccgtcctgtgccaggaccacggcctgaccccagaacaagttgtcgcgattgcaagcaacaacggaggcaaacaagccttagaaacagtccagagattgttgccggtgctgtgccaagcccacggcctgacccccgaccaggttgtcgctattgctagtaacggcggaggcaaacaggcgctggaaacagttcagcgcctcttgccggtcttgtgtcaggcccacggcctgaccccggcccaggtggttgcaatcgcgtcacacgatgggggaaagcaggccctagaaaccgttcagcgactcctgcccgtcctgtgccaggaccacggcctgaccccagaccaagttgtcgcgattgcaagcaacaacggaggcaaacaagccttagaaacagtccagagattgttgccggtgctgtgccaagaccacggcctgaccccagaacaggttgtggccatcgccagcaacataggtggcaagcaggccctcgaaaccgtccagagactgttaccggttctctgccaggcccacggcctgaccccggaccaggtggttgcaatcgcgtcacacgatgggggaaagcaggccctagaaaccgttcagcgactcctgcccgtcctgtgccaggcccacggcctgacccccgcccaggttgtcgctattgctagtaacggcggaggcaaacaggcgctggaaacagttcagcgcctcttgccggtcttgtgtcaggaccacggcctgaccccggaccaggtggttgcaatcgcgtcacacgatgggggaaagcaggccctagaaaccgttcagcgactcctgcccgtcctgtgccaggaccacggcctgaccccagaacaagttgtcgcgattgcaagcaacaacggaggcaaacaagccttagaaacagtccagagattgttgccggtgctgtgccaagcccacggcctgaccccagaccaagttgtcgcgattgcaagcaacaacggaggcaaacaagccttagaaacagtccagagattgttgcctgtgctgtgccaagcccacggcctgaccccggcccaggtggttgcaatcgcgtcacacgatgggggaaagcaggccctagaaaccgttcagcgactcctgcccgtcctgtgccaggaccacggcctgaccccagaccaagttgtcgcgattgcaagcaacaacggaggcaaacaagccttagaaacagtccagagattgttgccggtgctgtgccaagaccacggcctgaccccagaacaagttgtcgcgattgcaagcaacaacggaggcaaacaagccttagaaacagtccagagattgttgccggtgctgtgccaagcccacggcctgaccccagaccaagttgtcgcgattgcaagcaacaacggaggcaaacaagccttagaaacagtccagagattgttgcctgtgctgtgccaagcccacggcctgaccccagcccaagttgtcgcgattgcaagcaacaacggaggcaaacaagccttagaaacagtccagagattgttgccggtgctgtgccaagaccacggcctgacccccgaacaggtcgtcgccatcgcctctaacggtggtggccgacccgccctcgaatccatcgtggcgcagctctctcgacccgatcccgccttggccgccctcacgaatgaccacctcgtcgccctcgcctgtttgggcggtcgacccgccatggacgcggtcaagaagggcctccctcacgcccctgagctcatccgctcccagctcgtcaagtccgaactcgaggagaagaagtccgagctccgacacaagttgaagtacgtcccccacgagtacatcgagttgatcgagattgcccgcaactccacccaggaccgcatcctcgagatgaaggtcatggagttttttatgaaagtctacggttaccgcggtaagcacctcggtggttcccgcaagcccgatggtgccatctatacggtgggttctcccatcgactacggtgtcatcgtggacaccaaggcgtactccggtggctacaacctccccatcggccaggccgacgagatgcaacgatatgtggaggagaaccagacccgcaacaagcacatcaaccccaacgagtggtggaaggtctacccttcctccgtcaccgagttcaagttcttgtttgtttctggtcatttcaagggtaactacaaggcccaactcacccgactcaaccacatcaccaactgcaacggcgccgtcctctccgtcgaggagctcttgatcggcggcgaaatgatcaaggccggtaccctcaccctcgaggaggtccgccgcaagtttaacaacggcgagatcaacttttgagccgcagcctcttgggtgaagtgtttttaccccccttctccttcacccccgcattcagatgtgcagcgtaaccatacctgctatacataccttgcatcatctagaataactagaaggtcaacgacaatatcttaaaactgagattttgaacgaaagagacttaacaaacagtaggaaataggaagtaatatggaagggatacagctagtagcaaatgattgagtctaagtcctgtcgtttggttcgtgcccgcccctcgtttacatcaagaaatgaaattctcgtcagacagcaggagggagaacattcaccgttaaaagcgtgtagcctttccagagatagagatggaaaagcaagcgacctatcagccgatgaaataatttaaaaagaaaagaaagaaaaggtaacgaggattcaataattgctctgatcctacctagtcgatgataatcttgtctctccttattcttttcggttgtattaatcgcccaatctgaataatgttacaaccaattaaccaattctgattagaaaaactcatcgagcatcaaatgaaactgcaatttattcatatcaggattatcaataccatatttttgaaaaagccgtttctgtaatgaaggagaaaactcaccgaggcagttccataggatggcaagatcctggtatcggtctgcgattccgactcgtccaacatcaatacaacctattaatttcccctcgtcaaaaataaggttatcaagtgagaaatcaccatgagtgacgactgaatccggtgagaatggcaaaagtttatgcatttctttccagacttgttcaacaggccagccattacgctcgtcatcaaaatcactcgcatcaaccaaaccgttattcattcgtgattgcgcctgagcaaggcgaaatacgcgatcgctgttaaaaggacaattacaaacaggaatcgaatgcaaccggcgcagggacactgccagcgcatcaacaatattttcacctgaatcaggatattcttctaatacctggaatgctgtttttccggggatcgcagtggtgagtaaccatgcatcatcaggagtacggataaaatgcttgatggtcggaagaggcataaattccgtcagccagtttagtctgaccatctcatctgtaacatcattggcaacgctacctttgccatgtttcagaaacaactctggcgcatcgggcttcccatacaagcgatagattgtcgcacctgattgcccgacattatcgcgagcccatttatacccatataaatcagcatccatgttggaatttaatcgcggcctcgacgtttcccgttgaatatggctcataacaccccttgtattactgtttatgtaagcagacagttttattgttcatgatgatatatttttatcttgtgcaatgtaacatcagagattttgagacacgggccagagctgcgtaccgagctcgaattcacgatgcggtattttctccttacgcatctgtgcggtatttcacaccaagtgccacctgggtccttttcatcacgtgctataaaaataattataatttaaattttttaatataaatatataaattaaaaatagaaagtaaaaaaagaaattaaagaaaaaatagtttttgttttccgaagatgtaaaagactctagggggatcgccaacaaatactaccttttatcttgctcttcctgctctcaggtattaatgccgaattgtttcatcttgtctgtgtagaagaccacacacgaaaatcctgtgattttacattttacttatcgttaatcgaatgtatatctatttaatctgcttttcttgtctaataaatatatatgtaaagtacgctttttgttgaaattttttaaacctttgtttatttttttttcttcattccgtaactcttctaccttctttatttactttctaaaatccaaatacaaaacataaaaataaataaacacagagtaaattcccaaattattccatcattaaaagatacgaggcgcgtgtaagttacaggcaagcgatcccaaaaggccaggaaccgtaaaaaggccgcgttgctggcgtttttccataggctccgcccccctgacgagcatcacaaaaatcgacgctcaagtcagaggtggcgaaacccgacaggactataaagataccaggcgtttccccctggaagctccctcgtgcgctctcctgttccgaccctgccgcttaccggatacctgtccgcctttctcccttcgggaagcgtggcgctttctcatagctcacgctgtaggtatctcagttcggtgtaggtcgttcgctccaagctgggctgtgtgcacgaaccccccgttcagcccgaccgctgcgccttatccggtaactatcgtcttgagtccaacccggtaagacacgacttatcgccactggcagcagccactggtaacaggattagcagagcgaggtatgtaggcggtgctacagagttcttgaagtggtggcctaactacggctacactagaagaacagtatttggtatctgcgctctgctgaagccagttaccttcggaaaaagagttggtagctcttgatccggcaaacaaaccaccgctggtagcggtggtttttttgtttgcaagcagcagattacgcgcagaaaaaaaggatctcaagaagatcctttgatcttttctacggggtctgacgctcagtggaacgaaaactcacgttaagggattttggtcatgagattatcaaaaaggatcttcacctagatccttttaaattaaaaatgaagttttaaatcaatctaaagtatatatgagtaaacttggtctgacagttaccaatgcttaatcagtgaggcacctatctcagcgatctgtctatttcgttcatccatagttgcctgactccccgtcgtgtagataactacgatacgggagggcttaccatctggccccagtgctgcaatgataccgcgagacccacgctcaccggctccagatttatcagcaataaaccagccagccggaagggccgagcgcagaagtggtcctgcaactttatccgcctccatccagtctattaattgttgccgggaagctagagtaagtagttcgccagttaatagtttgcgcaacgttgttgccattgctacaggcatcgtggtgtcacgctcgtcgtttggtatggcttcattcagctccggttcccaacgatcaaggcgagttacatgatcccccatgttgtgcaaaaaagcggttagctccttcggtcctccgatcgttgtcagaagtaagttggccgcagtgttatcactcatggttatggcagcactgcataattctcttactgtcatgccatccgtaagatgcttttctgtgactggtgagtactcaaccaagtcattctgagaatagtgtatgcggcgaccgagttgctcttgcccggcgtcaatacgggataataccgcgccacatagcagaactttaaaagtgctcatcattggaaaacgttcttcggggcgaaaactctcaaggatcttaccgctgttgagatccagttcgatgtaacccactcgtgcacccaactgatcttcagcatcttttactttcaccagcgtttctgggtgagcaaaaacaggaaggcaaaatgccgcaaaaaagggaataagggcgacacggaaatgttgaatactcatactcttcctttttcaatattattgaagcatttatcagggttattgtctcatgagcggatacatatttgaatgtatttagaaaaataaacaaataggggttccgcgcacatttccccgaaaagtgccacctgacgtctaagaaaccattattatcatgacattaacctataaaaataggcgtatcacgaggccctttcgtctggcgcgtttcggtgatgacggtgaaaacctctgacacatgcagctcccgatatcggtcacagcttgtctgtaagcggatgccgggagcagacaagcccgtcagggcgcgtcagcgggtgttggcgggtgtcgggatgaccatgattacgccaagctatttaggtgacactataggggaaagcttgcatgcctgcaggtcgactctagaggatctactagtcatatggattggtggagtgagatagcaggagcatcacgcctcacttacggcaaccagcaacagcaacacctgcttgaagcatcaccgcgaacacaggtatgcgcttatggaccttgaacgaatccatgctgcctcaagctcccctccttgcgtgccgtcttgcttgccttaacccttctgcagacgccctagacaagaaataagaggccatccaatagatgattacagatagtggagacccaaaatgctgcacatgcgaccttatttgccattcggggctgagaatcgtgcgcagcgtcgaagccttttttctgcctccctcctctccttccttggatcacttgcttcccattcgcatgtcctgcttgctgcttccctcccccagccaccctcaagtcaaggactttacttccttcttctcacatccaacacaggtgcaactccctccttctttcccaagcatggacgatgcgttgcgtgcactgcggggtcggtatcccggttgtgagtgggttgttgtggaggatggggcctcgggggctggtgtttatcggcttcggggtggtgggcgggagttgtttgtcaaggtggcagctctgggggccggggtgggcttgttgggtgaggctgagcggctggtgtggttggcggaggtggggattcccgtacctcgtgttgtggagggtggtggggacgagagggtcgcctggttggtcaccgaagcggttccggggcgtccggccagtgcgcggtggccgcgggagcagcggctggacgtggcggtggcgctcgcggggctcgctcgttcgctgcacgcgctggactgggagcggtgtccgttcgatcgcagtctcgcggtgacggtgtagtctggaacatgagcccgcaaggagaggacggcggccccgccgactcgacgattgttccgtccgccctccgcacaaggagtctggaacgtctctaagatggagtggatggaggaggaggcgagcgtagcagcaagcgtgagttatacagccaggcacatgtcgcaatccttcggtctcgggcttaaaatccacgcactaatcacgctgggccatgcaaagagcaatgccgaggcccaccacacaaaacgctgtgtcgcgcgttgcggcctgaagcttcatacttcttagtcgccgccaaaagggctcgagagacgagacccgttggcatgaccgatgttgttcgacgcggtttgcttcgtcacagtcgacgtgattcaggaatctggagcctgcagatcatttttttcagcctgatatcgttcttttccactgagaaccatcagaccaccttttcttccattgtgtgaaggagtaggagttgccgtgctgctttgtgggagacatctgcgatggtgaccagcctcccgtcgtctggtcgacgtgacgagcctcttcactgttcttcgacggagagacgcaagcgagacggctctagaccttttggacacgcattctgtgtgtgaactagtggacagtgataccacgtctgaaagctcaccactgcccatggtgcagctacttgtcacaaagttttgactccgtcggtatcaccattcgcgctcgtgtgcctggttgttccgccacgccggcctgccccggggcggggcaatattctaaaatctcacgcaaaacaccgcacttacccctcacacatattcgtgatagaccaccaccaatctcagcccgcatcaacaatgagcccgcaaggagaggacggcggccccgccgactctggaacatgagcccgcaaggagaggacggcggccccgccgactcgacgatagattcccgtacctcgtgttgtggagggtggtggggacgagagggtcgcctggttggtcaccgaagcggttccggggcgtccggccagtgcgcggtggccgcgggagcagcggctggacgtggcggtggcgctcgcggggctcgctcgttcgctgcacgcgctggactgggagcggtgtccgttcgatcgcagtctcgcggtgacggtgccgcaggcggcccgtgctgtcgctgaagggagcgtcgacttggaggatctggacgaggagcggaaggggtggtcgggggagcggcttctcgccgagctggagcggactcggcctgcggacgaggatctggcggtttgccacggtgacctgtgcccggacaacgtgctgctcgaccctcgtacctgcgaggtgaccgggctgatcgacgtggggcgggtcggccgtgcggaccggcactccgatctcgcgctggtgctgcgcgagctggcccacgaggaggacccgtggttcgggccggagtgttccgcggcgttcctgcgggagtacgggcgcgggtgggatggggcggtatcggaggaaaagctggcgttttaccggctgttggacgaatttttctgagccgcagcctcttgggtgaagtgtttttaccccccttctccttcacccccgcattcagatgtgcagcgtaaccatacctgctatacataccttgcatcatctagaataactagaaggtcaacgacaatatcttaaaactgagattttgaacgaaagagacttaacaaacagtaggaaataggaagtaatatggaagggatacagctagtagcaaatgattgagtctaagtcctgtcgtttggttcgtgcccgcccctcgtttacatcaagaaatgaaattctcgtcagacagcaggagggagaacattcaccgttaaaagcgtgtagcctttccagagatagagatggaaaagcaagcgacctatcagccgatgaaataatttaaaaagaaaagaaagaaaaggtaacgaggattcaataattgctctgatcctacctagtcgatgataatcttgtctctccttattcttttcggttgtatt

SEQ ID NO: 19 - DNA, 15133 bp, synthetic construct
  source 1..15133: mol_type = other DNA; note = all-in-one NICS210
ttcctgcgttatcccctgattctgtggataaccgtattaccgcctttgagtgagctgataccgctcgccgcagccgaacgaccgagcgcagcgagtcagtgagcgaggaagcggaagagcgcccaatacgcaaaccgcctctccccgcgcgttggccgattcattaatgcagctgcggccgcatgaccatgattacgccaagctatttaggtgacactataggggaaagcttgcatgcctgcaggtcgactctagaggatctactagtcatatggattggtggagtgagatagcaggagcatcacgcctcacttacggcaaccagcaacagcaacacctgcttgaagcatcaccgcgaacacaggtatgcgcttatggaccttgaacgaatccatgctgcctcaagctcccctccttgcgtgccgtcttgcttgccttaacccttctgcagacgccctagacaagaaataagaggccatccaatagatgattacagatagtggagacccaaaatgctgcacatgcgaccttatttgccattcggggctgagaatcgtgcgcagcgtcgaagccttttttctgcctccctcctctccttccttggatcacttgcttcccattcgcatgtcctgcttgctgcttccctcccccagccaccctcaagtcaaggactttacttccttcttctcacatccaacacaggtgcaactccctccttctttcccaagcatggcctcctccccccccaagaaaaagcgcaaggtcgccgccgccgattacaaggacgacgacgacaagtcctggaaagacgcgtccggttggtcccgaatgcatgccgcccctcgccgccgcgcggcccagccctccgacgcctcccccgccgcccaagtcgacctccgaaccttgggttactctcagcagcagcaggagaagatcaagcctaaggtccgctccaccgtcgcgcagcatcacgaggccctcgtcggccacggtttcacccatgcccacattgtggccctctcccagcatcccgccgccttgggcacggtggccgtgacgtaccagcacatcatcacggccctccccgaggccacccacgaggatatcgtgggtgtcggtaaacagtggtccggcgcccgcgccttggaggccctcctcaccgatgccggcgaactccgaggtcctcctctccaactcgacaccggccagttggtcaagattgccaagcgcggcggtgtcaccgccatggaggccgtccatgcgtcccgcaacgccttgaccggcgcccccctcaacctgaccccggaccaggtggttgcaatcgcgtcacacgatgggggaaagcaggccctagaaaccgttcagcgactcctgcccgtcctgtgccaggaccacggcctgacccccgaacaggttgtcgctattgctagtaacggcggaggcaaacaggcgctggaaacagttcagcgcctcttgccggtcttgtgtcaggcccacggcctgaccccagaccaagttgtcgcgattgcaagcaacaacggaggcaaacaagccttagaaacagtccagagattgttgcctgtgctgtgccaagcccacggcctgaccccagcccaagttgtcgcgattgcaagcaacaacggaggcaaacaagccttagaaacagtccagagattgttgccggtgctgtgccaagaccacggcctgaccccagaccaggttgtggccatcgccagcaacataggtggcaagcaggccctcgaaaccgtccagagactgttaccggttctctgccaggaccacggcctgaccccagaacaggttgtggccatcgccagcaacataggtggcaagcaggccctcgaaaccgtccagagactgttaccggttctctgccaggcccacggcctgaccccggaccaggtggttgcaatcgcgtcacacgatgggggaaagcaggccctagaaaccgttcagcgactcctgcccgtcctgtgccaggcccacggcctgaccccagcccaggttgtggccatcgccagcaacataggtggcaagcaggccctcgaaaccgtccagagactgttaccggttctctgccaggaccacggcctgacccccgaccaggttgtcgctattgctagtaacggcggaggcaaacaggcgctggaaacagttcagcgcctcttgccggtcttgtgtcaggaccacggcctgaccccagaacaagttgtcgcgattgcaagcaacaacggaggcaaacaagccttagaaacagtccagagattgttgccggtgctgtgccaagcccacggcctgaccccagaccaggttgtggccatcgccagcaacataggtggcaagcaggccctcgaaaccgtccagagactgttaccggttctctgccaggcccacggcctgaccccagcccaagttgtcgcgattgcaagcaacaacggaggcaaacaagccttagaaacagtccagagattgttgccggtgctgtgccaagaccacggcctgaccccggaccaggtggttgcaatcgcgtcacacgatgggggaaagcaggccctagaaaccgttcagcgactcctgcccgtcctgtgccaggaccacggcctgaccccggaacaggtggttgcaatcgcgtcacacgatgggggaaagcaggccctagaaaccgttcagcgactcctgcccgtcctgtgccaggcccacggcctgaccccggaccaggtggttgcaatcgcgtcacacgatgggggaaagcaggccctagaaaccgttcagcgactcctgcccgtcctgtgccaggcccacggcctgaccccagcccaagttgtcgcgattgcaagcaacaacggaggcaaacaagccttagaaacagtccagagattgttgccggtgctgtgccaagaccacggcctgacccccgaacaggtcgtcgccatcgcctctaacggtggtggccgacccgccctcgaatccatcgtggcgcagctctctcgacccgatcccgccttggccgccctcacgaatgaccacctcgtcgccctcgcctgtttgggcggtcgacccgccatggacgcggtcaagaagggcctccctcacgcccctgagctcatccgctcccagctcgtcaagtccgaactcgaggagaagaagtccgagctccgacacaagttgaagtacgtcccccacgagtacatcgagttgatcgagattgcccgcaactccacccaggaccgcatcctcgagatgaaggtcatggagttttttatgaaagtctacggttaccgcggtaagcacctcggtggttcccgcaagcccgatggtgccatctatacggtgggttctcccatcgactacggtgtcatcgtggacaccaaggcgtactccggtggctacaacctccccatcggccaggccgacgagatgcaacgatatgtggaggagaaccagacccgcaacaagcacatcaaccccaacgagtggtggaaggtctacccttcctccgtcaccgagttcaagttcttgtttgtttctggtcatttcaagggtaactacaaggcccaactcacccgactcaaccacatcaccaactgcaacggcgccgtcctctccgtcgaggagctcttgatcggcggcgaaatgatcaaggccggtaccctcaccctcgaggaggtccgccgcaagtttaacaacggcgagatcaacttttgagccgcagcctcttgggtgaagtgtttttaccccccttctccttcacccccgcattcagatgtgcagcgtaaccatacctgctatacataccttgcatcatctagaataactagaaggtcaacgacaatatcttaaaactgagattttgaacgaaagagacttaacaaacagtaggaaataggaagtaatatggaagggatacagctagtagcaaatgattgagtctaagtcctgtcgtttggttcgtgcccgcccctcgtttacatcaagaaatgaaattctcgtcagacagcaggagggagaacattcaccgttaaaagcgtgtagcctttccagagatagagatggaaaagcaagcgacctatcagccgatgaaataatttaaaaagaaaagaaagaaaaggtaacgaggattcaataattgctctgatcctacctagtcgatgataatcttgtctctccttattcttttcggttgtattaatcgggatccatgaccatgattacgccaagctatttaggtgacactataggggaaagcttgcatgcctgcaggtcgactctagaggatctactagtcatatggattggtggagtgagatagcaggagcatcacgcctcacttacggcaaccagcaacagcaacacctgcttgaagcatcaccgcgaacacaggtatgcgcttatggaccttgaacgaatccatgctgcctcaagctcccctccttgcgtgccgtcttgcttgccttaacccttctgcagacgccctagacaagaaataagaggccatccaatagatgattacagatagtggagacccaaaatgctgcacatgcgaccttatttgccattcggggctgagaatcgtgcgcagcgtcgaagccttttttctgcctccctcctctccttccttggatcacttgcttcccattcgcatgtcctgcttgctgcttccctcccccagccaccctcaagtcaaggactttacttccttcttctcacatccaacacaggtgcaactccctccttctttcccaagcatggcctcctccccccccaagaaaaagcgcaaggtcgccgccgccgattacaaggacgacgacgacaagtcctggaaagacgcgtccggttggtcccgaatgcatgccgcccctcgccgccgcgcggcccagccctccgacgcctcccccgccgcccaagtcgacctccgaaccttgggttactctcagcagcagcaggagaagatcaagcctaaggtccgctccaccgtcgcgcagcatcacgaggccctcgtcggccacggtttcacccatgcccacattgtggccctctcccagcatcccgccgccttgggcacggtggccgtgacgtaccagcacatcatcacggccctccccgaggccacccacgaggatatcgtgggtgtcggtaaacagtggtccggcgcccgcgccttggaggccctcctcaccgatgccggcgaactccgaggtcctcctctccaactcgacaccggccagttggtcaagattgccaagcgcggcggtgtcaccgccatggaggccgtccatgcgtcccgcaacgccttgaccggcgcccccctcaacctgaccccggaccaggtggttgcaatcgcgtcacacgatgggggaaagcaggccctagaaaccgttcagcgactcctgcccgtcctgtgccaggaccacggcctgaccccagaacaagttgtcgcgattgcaagcaacaacggaggcaaacaagccttagaaacagtccagagattgttgccggtgctgtgccaagcccacggcctgacccccgaccaggttgtcgctattgctagtaacggcggaggcaaacaggcgctggaaacagttcagcgcctcttgccggtcttgtgtcaggcccacggcctgaccccggcccaggtggttgcaatcgcgtcacacgatgggggaaagcaggccctagaaaccgttcagcgactcctgcccgtcctgtgccaggaccacggcctgaccccagaccaagttgtcgcgattgcaagcaacaacggaggcaaacaagccttagaaacagtccagagattgttgccggtgctgtgccaagaccacggcctgaccccagaacaggttgtggccatcgccagcaacataggtggcaagcaggccctcgaaaccgtccagagactgttaccggttctctgccaggcccacggcctgaccccggaccaggtggttgcaatcgcgtcacacgatgggggaaagcaggccctagaaaccgttcagcgactcctgcccgtcctgtgccaggcccacggcctgacccccgcccaggttgtcgctattgctagtaacggcggaggcaaacaggcgctggaaacagttcagcgcctcttgccggtcttgtgtcaggaccacggcctgaccccggaccaggtggttgcaatcgcgtcacacgatgggggaaagcaggccctagaaaccgttcagcgactcctgcccgtcctgtgccaggaccacggcctgaccccagaacaagttgtcgcgattgcaagcaacaacggaggcaaacaagccttagaaacagtccagagattgttgccggtgctgtgccaagcccacggcctgaccccagaccaagttgtcgcgattgcaagcaacaacggaggcaaacaagccttagaaacagtccagagattgttgcctgtgctgtgccaagcccacggcctgaccccggcccaggtggttgcaatcgcgtcacacgatgggggaaagcaggccctagaaaccgttcagcgactcctgcccgtcctgtgccaggaccacggcctgaccccagaccaagttgtcgcgattgcaagcaacaacggaggcaaacaagccttagaaacagtccagagattgttgccggtgctgtgccaagaccacggcctgaccccagaacaagttgtcgcgattgcaagcaacaacggaggcaaacaagccttagaaacagtccagagattgttgccggtgctgtgccaagcccacggcctgaccccagaccaagttgtcgcgattgcaagcaacaacggaggcaaacaagccttagaaacagtccagagattgttgcctgtgctgtgccaagcccacggcctgaccccagcccaagttgtcgcgattgcaagcaacaacggaggcaaacaagccttagaaacagtccagagattgttgccggtgctgtgccaagaccacggcctgacccccgaacaggtcgtcgccatcgcctctaacggtggtggccgacccgccctcgaatccatcgtggcgcagctctctcgacccgatcccgccttggccgccctcacgaatgaccacctcgtcgccctcgcctgtttgggcggtcgacccgccatggacgcggtcaagaagggcctccctcacgcccctgagctcatccgctcccagctcgtcaagtccgaactcgaggagaagaagtccgagctccgacacaagttgaagtacgtcccccacgagtacatcgagttgatcgagattgcccgcaactccacccaggaccgcatcctcgagatgaaggtcatggagttttttatgaaagtctacggttaccgcggtaagcacctcggtggttcccgcaagcccgatggtgccatctatacggtgggttctcccatcgactacggtgtcatcgtggacaccaaggcgtactccggtggctacaacctccccatcggccaggccgacgagatgcaacgatatgtggaggagaaccagacccgcaacaagcacatcaaccccaacgagtggtggaaggtctacccttcctccgtcaccgagttcaagttcttgtttgtttctggtcatttcaagggtaactacaaggcccaactcacccgactcaaccacatcaccaactgcaacggcgccgtcctctccgtcgaggagctcttgatcggcggcgaaatgatcaaggccggtaccctcaccctcgaggaggtccgccgcaagtttaacaacggcgagatcaacttttgagccgcagcctcttgggtgaagtgtttttaccccccttctccttcacccccgcattcagatgtgcagcgtaaccatacctgctatacataccttgcatcatctagaataactagaaggtcaacgacaatatcttaaaactgagattttgaacgaaagagacttaacaaacagtaggaaataggaagtaatatggaagggatacagctagtagcaaatgattgagtctaagtcctgtcgtttggttcgtgcccgcccctcgtttacatcaagaaatgaaattctcgtcagacagcaggagggagaacattcaccgttaaaagcgtgtagcctttccagagatagagatggaaaagcaagcgacctatcagccgatgaaataatttaaaaagaaaagaaagaaaaggtaacgaggattcaataattgctctgatcctacctagtcgatgataatcttgtctctccttattcttttcggttgtattaatcgcccaatctgaataatgttacaaccaattaaccaattctgattagaaaaactcatcgagcatcaaatgaaactgcaatttattcatatcaggattatcaataccatatttttgaaaaagccgtttctgtaatgaaggagaaaactcaccgaggcagttccataggatggcaagatcctggtatcggtctgcgattccgactcgtccaacatcaatacaacctattaatttcccctcgtcaaaaataaggttatcaagtgagaaatcaccatgagtgacgactgaatccggtgagaatggcaaaagtttatgcatttctttccagacttgttcaacaggccagccattacgctcgtcatcaaaatcactcgcatcaaccaaaccgttattcattcgtgattgcgcctgagcaaggcgaaatacgcgatcgctgttaaaaggacaattacaaacaggaatcgaatgcaaccggcgcagggacactgccagcgcatcaacaatattttcacctgaatcaggatattcttctaatacctggaatgctgtttttccggggatcgcagtggtgagtaaccatgcatcatcaggagtacggataaaatgcttgatggtcggaagaggcataaattccgtcagccagtttagtctgaccatctcatctgtaacatcattggcaacgctacctttgccatgtttcagaaacaactctggcgcatcgggcttcccatacaagcgatagattgtcgcacctgattgcccgacattatcgcgagcccatttatacccatataaatcagcatccatgttggaatttaatcgcggcctcgacgtttcccgttgaatatggctcataacaccccttgtattactgtttatgtaagcagacagttttattgttcatgatgatatatttttatcttgtgcaatgtaacatcagagattttgagacacgggccagagctgcgtaccgagctcgaattcacgatgcggtattttctccttacgcatctgtgcggtatttcacaccaagtgccacctgggtccttttcatcacgtgctataaaaataattataatttaaattttttaatataaatatataaattaaaaatagaaagtaaaaaaagaaattaaagaaaaaatagtttttgttttccgaagatgtaaaagactctagggggatcgccaacaaatactaccttttatcttgctcttcctgctctcaggtattaatgccgaattgtttcatcttgtctgtgtagaagaccacacacgaaaatcctgtgattttacattttacttatcgttaatcgaatgtatatctatttaatctgcttttcttgtctaataaatatatatgtaaagtacgctttttgttgaaattttttaaacctttgtttatttttttttcttcattccgtaactcttctaccttctttatttactttctaaaatccaaatacaaaacataaaaataaataaacacagagtaaattcccaaattattccatcattaaaagatacgaggcgcgtgtaagttacaggcaagcgatcccaaaaggccaggaaccgtaaaaaggccgcgttgctggcgtttttccataggctccgcccccctgacgagcatcacaaaaatcgacgctcaagtcagaggtggcgaaacccgacaggactataaagataccaggcgtttccccctggaagctccctcgtgcgctctcctgttccgaccctgccgcttaccggatacctgtccgcctttctcccttcgggaagcgtggcgctttctcatagctcacgctgtaggtatctcagttcggtgtaggtcgttcgctccaagctgggctgtgtgcacgaaccccccgttcagcccgaccgctgcgccttatccggtaactatcgtcttgagtccaacccggtaagacacgacttatcgccactggcagcagccactggtaacaggattagcagagcgaggtatgtaggcggtgctacagagttcttgaagtggtggcctaactacggctacactagaagaacagtatttggtatctgcgctctgctgaagccagttaccttcggaaaaagagttggtagctcttgatccggcaaacaaaccaccgctggtagcggtggtttttttgtttgcaagcagcagattacgcgcagaaaaaaaggatctcaagaagatcctttgatcttttctacggggtctgacgctcagtggaacgaaaactcacgttaagggattttggtcatgagattatcaaaaaggatcttcacctagatccttttaaattaaaaatgaagttttaaatcaatctaaagtatatatgagtaaacttggtctgacagttaccaatgcttaatcagtgaggcacctatctcagcgatctgtctatttcgttcatccatagttgcctgactccccgtcgtgtagataactacgatacgggagggcttaccatctggccccagtgctgcaatgataccgcgagacccacgctcaccggctccagatttatcagcaataaaccagccagccggaagggccgagcgcagaagtggtcctgcaactttatccgcctccatccagtctattaattgttgccgggaagctagagtaagtagttcgccagttaatagtttgcgcaacgttgttgccattgctacaggcatcgtggtgtcacgctcgtcgtttggtatggcttcattcagctccggttcccaacgatcaaggcgagttacatgatcccccatgttgtgcaaaaaagcggttagctccttcggtcctccgatcgttgtcagaagtaagttggccgcagtgttatcactcatggttatggcagcactgcataattctcttactgtcatgccatccgtaagatgcttttctgtgactggtgagtactcaaccaagtcattctgagaatagtgtatgcggcgaccgagttgctcttgcccggcgtcaatacgggataataccgcgccacatagcagaactttaaaagtgctcatcattggaaaacgttcttcggggcgaaaactctcaaggatcttaccgctgttgagatccagttcgatgtaacccactcgtgcacccaactgatcttcagcatcttttactttcaccagcgtttctgggtgagcaaaaacaggaaggcaaaatgccgcaaaaaagggaataagggcgacacggaaatgttgaatactcatactcttcctttttcaatattattgaagcatttatcagggttattgtctcatgagcggatacatatttgaatgtatttagaaaaataaacaaataggggttccgcgcacatttccccgaaaagtgccacctgacgtctaagaaaccattattatcatgacattaacctataaaaataggcgtatcacgaggccctttcgtctggcgcgtttcggtgatgacggtgaaaacctctgacacatgcagctcccgatatcggtcacagcttgtctgtaagcggatgccgggagcagacaagcccgtcagggcgcgtcagcgggtgttggcgggtgtcgggatgaccatgattacgccaagctatttaggtgacactataggggaaagcttgcatgcctgcaggtcgactctagaggatctactagtcatatggattggtggagtgagatagcaggagcatcacgcctcacttacggcaaccagcaacagcaacacctgcttgaagcatcaccgcgaacacaggtatgcgcttatggaccttgaacgaatccatgctgcctcaagctcccctccttgcgtgccgtcttgcttgccttaacccttctgcagacgccctagacaagaaataagaggccatccaatagatgattacagatagtggagacccaaaatgctgcacatgcgaccttatttgccattcggggctgagaatcgtgcgcagcgtcgaagccttttttctgcctccctcctctccttccttggatcacttgcttcccattcgcatgtcctgcttgctgcttccctcccccagccaccctcaagtcaaggactttacttccttcttctcacatccaacacaggtgcaactccctccttctttcccaagcatggacgatgcgttgcgtgcactgcggggtcggtatcccggttgtgagtgggttgttgtggaggatggggcctcgggggctggtgtttatcggcttcggggtggtgggcgggagttgtttgtcaaggtggcagctctgggggccggggtgggcttgttgggtgaggctgagcggctggtgtggttggcggaggtggggattcccgtacctcgtgttgtggagggtggtggggacgagagggtcgcctggttggtcaccgaagcggttccggggcgtccggccagtgcgcggtggccgcgggagcagcggctggacgtggcggtggcgctcgcggggctcgctcgttcgctgcacgcgctggactgggagcggtgtccgttcgatcgcagtctcgcggtgacggtgtagtctggaacatgagcccgcaaggagaggacggcggccccgccgactcgacgaccatacacgttgaacatgaacatcaggtctcttatcttcttgctcactcaccactctgctccccatacactctcttcaccaacgaaaccttgtgcaggacacggtgttgttgtcaaggtcatagcatattaaagaagaccgacggcacaaccgtccgcttaggtggtttctgcgttgttccgtccgccctccgcacaaggagtctggaacgtctctaagatggagtggatggaggaggaggcgagcgtagcagcaagcgtgagttatacagccaggcacatgtcgcaatccttcggtctcgggcttaaaatccacgcactaatcacgctgggccatgcaaagagcaatgccgaggcccaccacacaaaacgctgtgtcgcgcgttgcggcctgaagcttcatacttcttagtcgccgccaaaagggctcgagagacgagacccgttggcatgaccgatgttgttcgacgcggtttgcttcgtcacagtcgacgtgattcaggaatctggagcctgcagatcatttttttcagcctgatatcgttcttttccactgagaaccatcagaccaccttttcttccattgtgtgaaggagtaggagttgccgtgctgctttgtgggagacatctgcgatggtgaccagcctcccgtcgtctggtcgacgtgacgagcctcttcactgttcttcgacggagagacgcaagcgagacggctctagaccttttggacacgcattctgtgtgtgaactagtggacagtgataccacgtctgaaagctcaccactgcccatggtgcagctacttgtcacaaagttttgactccgtcggtatcaccattcgcgctcgtgtgcctggttgttccgccacgccggcctgccccggggcggggcaatattctaaaatctcacgcaaaacaccgcacttacccctcacacatattcgtgatagaccaccaccaatctcagcccgcatcaacaatgagcccgcaaggagaggacggcggccccgccgactcgacgacgacgaggacgacgacgtctgaggcgatggccatgccggcaggagcagcagggacagcagccacatctgcatcagacagtcctagcagtcaccaagatgaagggggtggtcctacccaaacggtccaccgcgggccacacccggacattcacgaccagggggacaagtctggaacatgagcccgcaaggagaggacggcggccccgccgactcgacgatagattcccgtacctcgtgttgtggagggtggtggggacgagagggtcgcctggttggtcaccgaagcggttccggggcgtccggccagtgcgcggtggccgcgggagcagcggctggacgtggcggtggcgctcgcggggctcgctcgttcgctgcacgcgctggactgggagcggtgtccgttcgatcgcagtctcgcggtgacggtgccgcaggcggcccgtgctgtcgctgaagggagcgtcgacttggaggatctggacgaggagcggaaggggtggtcgggggagcggcttctcgccgagctggagcggactcggcctgcggacgaggatctggcggtttgccacggtgacctgtgcccggacaacgtgctgctcgaccctcgtacctgcgaggtgaccgggctgatcgacgtggggcgggtcggccgtgcggaccggcactccgatctcgcgctggtgctgcgcgagctggcccacgaggaggacccgtggttcgggccggagtgttccgcggcgttcctgcgggagtacgggcgcgggtgggatggggcggtatcggaggaaaagctggcgttttaccggctgttggacgaatttttctgagccgcagcctcttgggtgaagtgtttttaccccccttctccttcacccccgcattcagatgtgcagcgtaaccatacctgctatacataccttgcatcatctagaataactagaaggtcaacgacaatatcttaaaactgagattttgaacgaaagagacttaacaaacagtaggaaataggaagtaatatggaagggatacagctagtagcaaatgattgagtctaagtcctgtcgtttggttcgtgcccgcccctcgtttacatcaagaaatgaaattctcgtcagacagcaggagggagaacattcaccgttaaaagcgtgtagcctttccagagatagagatggaaaagcaagcgacctatcagccgatgaaataatttaaaaagaaaagaaagaaaaggtaacgaggattcaataattgctctgatcctacctagtcgatgataatcttgtctctccttattcttttcggttgtatt

SEQ ID NO: 20 - DNA, 1304 bp, synthetic construct
  source 1..1304: mol_type = other DNA; note = knock in fragment
ttgctgtgtggttcttcacgtcctccgtcctttctctttgtaatcatgcagtcgcccacttactggctcgcccccccgtcgcttttccacgctacagccacccaccaaatcacaggacgggcttcgattcgacacatcgaatcaaaggaggatacttctcccaggctgtcgctcttgctgtaggttgccgttgccgtgggccccccttaaaagccgcgtctctaagatggagtggatggaggaggaggcgagcgtagcagcaagcgtgagttatacagccaggcacatgtcgcaatccttcggtctcgggcttaaaatccacgcactaatcacgctgggccatgcaaagagcaatgccgaggcccaccacacaaaacgctgtgtcgcgcgttgcggcctgaagcttcatacttcttagtcgccgccaaaagggctcgagagacgagacccgttggcatgaccgatgttgttcgacgcggtttgcttcgtcacagtcgacgtgattcaggaatctggagcctgcagatcatttttttcagcctgatatcgttcttttccactgagaaccatcagaccaccttttcttccattgtgtgaaggagtaggagttgccgtgctgctttgtgggagacatctgcgatggtgaccagcctcccgtcgtctggtcgacgtgacgagcctcttcactgttcttcgacggagagacgcaagcgagacggctctagaccttttggacacgcattctgtgtgtgaactagtggacagtgataccacgtctgaaagctcaccactgcccatggtgcagctacttgtcacaaagttttgactccgtcggtatcaccattcgcgctcgtgtgcctggttgttccgccacgccggcctgccccggggcggggcaatattctaaaatctcacgcaaaacaccgcacttacccctcacacatattcgtgatagaccaccaccaatctcagcccgcatcaacaatggggacgccaacaacgccgtccacgccccaacgaaatggtgagcggctcgagacccgacccttggacacgtcgagcgacaaagtaaatggtggcgccggcggcagcaaaacccatgaggtctcggcatccatctcggccgatttattaggctacttcctcgcggtactcattctcctaaacttctggtcggccgcatttttggaactagtcatgtacgtggtgtttgcgccgatgtatccaccaatatggcacgcaacccgcatccttggcgttcgcttcggctggctcccccctatgatcttcctcaagtgggccaa

SEQ ID NO: 21 - DNA, 1239 bp, Nannochloropsis oceanica
  source 1..1239: mol_type = genomic DNA
atggggacgccaacaacgccgtccacgccccaacgaaatggtgagcggctcgagacccgacccttggacacgtcgagcgacaaagtaaatggtggcgccggcggcagcaaaacccatgaggtctcggcttccatttcggcggatttattaggctacttcctcgcggtactcattctcctaaacttctggtcggccgcatttttggaactagtcatgtacgtggtgtttgcgccgatgtatccaccaatatggcacgcaacccgcatccttggcgttcgcttcggctggctcccccctatgatcttcctcaagtgggccaacattcgactgcgggtcacagggcacgctgcagcagcttctggcctggggaccatgccttcttcttcctcctcctcctggtcctcgtcatggcaacggtacatcgaccttttcacccccggcaagcttccccgtgccttgatcatgatcaaccacctctcgtgggcagattccttcgtcctctccccttggctgcatgcccacaacagcgtcaacggcgatacctgttggccaatgtggcgggggttcatcaacatgcccttgggatggattgcctacatgtcagaatgccctgttttagggtacgggaaagagatggacctcgagacaatccgcaagagcgtttcgcgtttttttcaacggaggatgacgaagtttttcctcttccccgagggcgccgtttttcgggaatgtatgcttcagaaatcccacgaatacgcccaagctaacaaccttcccctgctcgatcactgcctgctgccaaagcacggtgccttcctcgaggctggccaagcgctgcatcggcagggaatggagacactagtggacataaccattgcctaccccccaacttcctccctgtacaatgcacctttcaatgtcatagacttggtcaaatatcatccaacgccactgtatgtgcatttgaatgtgcggacgttcgatatgcgggagatcccctgggaggaggaggataaggtgcggcagtggcttacgcgtcggtttgaagagaaggatcgtttcttggacgattactacaagggaaagggaggggtgatggtggagggggggaaggaggaagggccccgatggagagatttggcattggatgtactgctgtggatgggggtacaagtggtcatgtatacagtgttgtacgcgctgggggcgagggtgctggggaggatgacggtgaggtga

SEQ ID NO: 22 - DNA, 27 bp, synthetic construct
  source 1..27: mol_type = other DNA; note = out-out-F1
atctccttcagcccctgcatgtagttc

SEQ ID NO: 23 - DNA, 25 bp, synthetic construct
  source 1..25: mol_type = other DNA; note = out-out-R1
actccttctcacctcaccgtcatcc

SEQ ID NO: 24 - DNA, 24 bp, synthetic construct
  source 1..24: mol_type = other DNA; note = 5'-R1
ggtctcgtctctcgagcccttttg

SEQ ID NO: 25 - DNA, 25 bp, synthetic construct
  source 1..25: mol_type = other DNA; note = 3'-F1
gacggctctagaccttttggacacg

SEQ ID NO: 26 - DNA, 25 bp, synthetic construct
  source 1..25: mol_type = other DNA; note = out-out-F2
ggggaaggaaaaagtgagctcgttc

SEQ ID NO: 27 - DNA, 25 bp, synthetic construct
  source 1..25: mol_type = other DNA; note = out-out- R2
ttccaggacggtaatgtcgatgttg

SEQ ID NO: 28 - DNA, 27 bp, synthetic construct
  source 1..27: mol_type = other DNA; note = 5'-R2
tcctcctccatccactccatcttagag

SEQ ID NO: 29 - DNA, 26 bp, synthetic construct
  source 1..26: mol_type = other DNA; note = 3'-F2
tcgtgatagaccaccaccaatctcag

SEQ ID NO: 30 - DNA, 50 bp, synthetic construct
  source 1..50: mol_type = other DNA
tccgttccacgcccaggcaacaaaactatgccgtctcgcagcaccatcga

SEQ ID NO: 31 - DNA, 17 bp, synthetic construct
  source 1..17: mol_type = other DNA
tccgttccacgcccagg

SEQ ID NO: 32 - DNA, 18 bp, synthetic construct
  source 1..18: mol_type = other DNA
gtctcgcagcaccatcga

SEQ ID NO: 33 - DNA, 200 bp, synthetic construct
  source 1..200: mol_type = other DNA
ctgggcttcgtaaatccatcagcactcacactgcctcccacataccatacacgatacacaggcacgcgtccggaggtgccggtgacggtaatttttctccgtgggactgtcggccatcgtaaggaacaaggccggcaaccaaggccaccagggcttattgcgaatcaagcacatccgttccacgcccaggcaacaaaact

SEQ ID NO: 34 - DNA, 208 bp, synthetic construct
  source 1..208: mol_type = other DNA
atgccgtctcgcagcaccatcgaggtcattaaggctgataagaaccagaacaatctggcgtatggcctaatcgttgtcattcttttggccattgatcccaagtaagtcattctgtcctcaaacatgccttgcttctttcaacacgacgacacggacacttcacactgagacacacgatgtgtgtctgcatgagtatgtaccgccttca

SEQ ID NO: 35 - DNA, 2895 bp, synthetic construct
  source 1..2895: mol_type = other DNA
atggcctcctccccccccaagaaaaagcgcaaggtcgccgccgccgattacaaggacgacgacgacaagtcctggaaagacgcgtccggttggtcccgaatgcatgccgcccctcgccgccgcgcggcccagccctccgacgcctcccccgccgcccaagtcgacctccgaaccttgggttactctcagcagcagcaggagaagatcaagcctaaggtccgctccaccgtcgcgcagcatcacgaggccctcgtcggccacggtttcacccatgcccacattgtggccctctcccagcatcccgccgccttgggcacggtggccgtgacgtaccagcacatcatcacggccctccccgaggccacccacgaggatatcgtgggtgtcggtaaacagtggtccggcgcccgcgccttggaggccctcctcaccgatgccggcgaactccgaggtcctcctctccaactcgacaccggccagttggtcaagattgccaagcgcggcggtgtcaccgccatggaggccgtccatgcgtcccgcaacgccttgaccggcgcccccctcaacctgaccccggaccaggtggttgcaatcgcgtcacacgatgggggaaagcaggccctagaaaccgttcagcgactcctgcccgtcctgtgccaggaccacggcctgaccccggaacaggtggttgcaatcgcgtcacacgatgggggaaagcaggccctagaaaccgttcagcgactcctgcccgtcctgtgccaggcccacggcctgaccccagaccaagttgtcgcgattgcaagcaacaacggaggcaaacaagccttagaaacagtccagagattgttgcctgtgctgtgccaagcccacggcctgacccccgcccaggttgtcgctattgctagtaacggcggaggcaaacaggcgctggaaacagttcagcgcctcttgccggtcttgtgtcaggaccacggcctgacccccgaccaggttgtcgctattgctagtaacggcggaggcaaacaggcgctggaaacagttcagcgcctcttgccggtcttgtgtcaggaccacggcctgaccccggaacaggtggttgcaatcgcgtcacacgatgggggaaagcaggccctagaaaccgttcagcgactcctgcccgtcctgtgccaggcccacggcctgaccccggaccaggtggttgcaatcgcgtcacacgatgggggaaagcaggccctagaaaccgttcagcgactcctgcccgtcctgtgccaggcccacggcctgaccccagcccaggttgtggccatcgccagcaacataggtggcaagcaggccctcgaaaccgtccagagactgttaccggttctctgccaggaccacggcctgaccccggaccaggtggttgcaatcgcgtcacacgatgggggaaagcaggccctagaaaccgttcagcgactcctgcccgtcctgtgccaggaccacggcctgaccccagaacaagttgtcgcgattgcaagcaacaacggaggcaaacaagccttagaaacagtccagagattgttgccggtgctgtgccaagcccacggcctgaccccggaccaggtggttgcaatcgcgtcacacgatgggggaaagcaggccctagaaaccgttcagcgactcctgcccgtcctgtgccaggcccacggcctgaccccggcccaggtggttgcaatcgcgtcacacgatgggggaaagcaggccctagaaaccgttcagcgactcctgcccgtcctgtgccaggaccacggcctgaccccggaccaggtggttgcaatcgcgtcacacgatgggggaaagcaggccctagaaaccgttcagcgactcctgcccgtcctgtgccaggaccacggcctgaccccagaacaggttgtggccatcgccagcaacataggtggcaagcaggccctcgaaaccgtccagagactgttaccggttctctgccaggcccacggcctgaccccagaccaagttgtcgcgattgcaagcaacaacggaggcaaacaagccttagaaacagtccagagattgttgcctgtgctgtgccaagcccacggcctgacccccgaacaggtcgtcgccatcgcctctaacggtggtggccgacccgccctcgaatccatcgtggcgcagctctctcgacccgatcccgccttggccgccctcacgaatgaccacctcgtcgccctcgcctgtttgggcggtcgacccgccatggacgcggtcaagaagggcctccctcacgcccctgagctcatccgctcccagctcgtcaagtccgaactcgaggagaagaagtccgagctccgacacaagttgaagtacgtcccccacgagtacatcgagttgatcgagattgcccgcaactccacccaggaccgcatcctcgagatgaaggtcatggagttttttatgaaagtctacggttaccgcggtaagcacctcggtggttcccgcaagcccgatggtgccatctatacggtgggttctcccatcgactacggtgtcatcgtggacaccaaggcgtactccggtggctacaacctccccatcggccaggccgacgagatgcaacgatatgtggaggagaaccagacccgcaacaagcacatcaaccccaacgagtggtggaaggtctacccttcctccgtcaccgagttcaagttcttgtttgtttctggtcatttcaagggtaactacaaggcccaactcacccgactcaaccacatcaccaactgcaacggcgccgtcctctccgtcgaggagctcttgatcggcggcgaaatgatcaaggccggtaccctcaccctcgaggaggtccgccgcaagtttaacaacggcgagatcaacttttga

SEQ ID NO: 36 - DNA, 2997 bp, synthetic construct
  source 1..2997: mol_type = other DNA
atggcctcctccccccccaagaaaaagcgcaaggtcgccgccgccgattacaaggacgacgacgacaagtcctggaaagacgcgtccggttggtcccgaatgcatgccgcccctcgccgccgcgcggcccagccctccgacgcctcccccgccgcccaagtcgacctccgaaccttgggttactctcagcagcagcaggagaagatcaagcctaaggtccgctccaccgtcgcgcagcatcacgaggccctcgtcggccacggtttcacccatgcccacattgtggccctctcccagcatcccgccgccttgggcacggtggccgtgacgtaccagcacatcatcacggccctccccgaggccacccacgaggatatcgtgggtgtcggtaaacagtggtccggcgcccgcgccttggaggccctcctcaccgatgccggcgaactccgaggtcctcctctccaactcgacaccggccagttggtcaagattgccaagcgcggcggtgtcaccgccatggaggccgtccatgcgtcccgcaacgccttgaccggcgcccccctcaacctgaccccggaccaggtggttgcaatcgcgtcacacgatgggggaaagcaggccctagaaaccgttcagcgactcctgcccgtcctgtgccaggaccacggcctgaccccagaacaagttgtcgcgattgcaagcaacaacggaggcaaacaagccttagaaacagtccagagattgttgccggtgctgtgccaagcccacggcctgaccccagaccaggttgtggccatcgccagcaacataggtggcaagcaggccctcgaaaccgtccagagactgttaccggttctctgccaggcccacggcctgacccccgcccaggttgtcgctattgctagtaacggcggaggcaaacaggcgctggaaacagttcagcgcctcttgccggtcttgtgtcaggaccacggcctgaccccagaccaagttgtcgcgattgcaagcaacaacggaggcaaacaagccttagaaacagtccagagattgttgccggtgctgtgccaagaccacggcctgaccccagaacaagttgtcgcgattgcaagcaacaacggaggcaaacaagccttagaaacagtccagagattgttgccggtgctgtgccaagcccacggcctgacccccgaccaggttgtcgctattgctagtaacggcggaggcaaacaggcgctggaaacagttcagcgcctcttgccggtcttgtgtcaggcccacggcctgaccccagcccaagttgtcgcgattgcaagcaacaacggaggcaaacaagccttagaaacagtccagagattgttgccggtgctgtgccaagaccacggcctgaccccggaccaggtggttgcaatcgcgtcacacgatgggggaaagcaggccctagaaaccgttcagcgactcctgcccgtcctgtgccaggaccacggcctgacccccgaacaggttgtcgctattgctagtaacggcggaggcaaacaggcgctggaaacagttcagcgcctcttgccggtcttgtgtcaggcccacggcctgaccccagaccaagttgtcgcgattgcaagcaacaacggaggcaaacaagccttagaaacagtccagagattgttgcctgtgctgtgccaagcccacggcctgaccccggcccaggtggttgcaatcgcgtcacacgatgggggaaagcaggccctagaaaccgttcagcgactcctgcccgtcctgtgccaggaccacggcctgaccccagaccaagttgtcgcgattgcaagcaacaacggaggcaaacaagccttagaaacagtccagagattgttgccggtgctgtgccaagaccacggcctgaccccagaacaggttgtggccatcgccagcaacataggtggcaagcaggccctcgaaaccgtccagagactgttaccggttctctgccaggcccacggcctgaccccagaccaagttgtcgcgattgcaagcaacaacggaggcaaacaagccttagaaacagtccagagattgttgcctgtgctgtgccaagcccacggcctgaccccagcccaggttgtggccatcgccagcaacataggtggcaagcaggccctcgaaaccgtccagagactgttaccggttctctgccaggaccacggcctgacccccgaacaggtcgtcgccatcgcctctaacggtggtggccgacccgccctcgaatccatcgtggcgcagctctctcgacccgatcccgccttggccgccctcacgaatgaccacctcgtcgccctcgcctgtttgggcggtcgacccgccatggacgcggtcaagaagggcctccctcacgcccctgagctcatccgctcccagctcgtcaagtccgaactcgaggagaagaagtccgagctccgacacaagttgaagtacgtcccccacgagtacatcgagttgatcgagattgcccgcaactccacccaggaccgcatcctcgagatgaaggtcatggagttttttatgaaagtctacggttaccgcggtaagcacctcggtggttcccgcaagcccgatggtgccatctatacggtgggttctcccatcgactacggtgtcatcgtggacaccaaggcgtactccggtggctacaacctccccatcggccaggccgacgagatgcaacgatatgtggaggagaaccagacccgcaacaagcacatcaaccccaacgagtggtggaaggtctacccttcctccgtcaccgagttcaagttcttgtttgtttctggtcatttcaagggtaactacaaggcccaactcacccgactcaaccacatcaccaactgcaacggcgccgtcctctccgtcgaggagctcttgatcggcggcgaaatgatcaaggccggtaccctcaccctcgaggaggtccgccgcaagtttaacaacggcgagatcaacttttga

SEQ ID NO: 37 - DNA, 15017 bp, synthetic construct
  source 1..15017: mol_type = other DNA
ttcctgcgttatcccctgattctgtggataaccgtattaccgcctttgagtgagctgataccgctcgccgcagccgaacgaccgagcgcagcgagtcagtgagcgaggaagcggaagagcgcccaatacgcaaaccgcctctccccgcgcgttggccgattcattaatgcagctgcggccgcatgaccatgattacgccaagctatttaggtgacactataggggaaagcttgcatgcctgcaggtcgactctagaggatctactagtcatatggattggtggagtgagatagcaggagcatcacgcctcacttacggcaaccagcaacagcaacacctgcttgaagcatcaccgcgaacacaggtatgcgcttatggaccttgaacgaatccatgctgcctcaagctcccctccttgcgtgccgtcttgcttgccttaacccttctgcagacgccctagacaagaaataagaggccatccaatagatgattacagatagtggagacccaaaatgctgcacatgcgaccttatttgccattcggggctgagaatcgtgcgcagcgtcgaagccttttttctgcctccctcctctccttccttggatcacttgcttcccattcgcatgtcctgcttgctgcttccctcccccagccaccctcaagtcaaggactttacttccttcttctcacatccaacacaggtgcaactccctccttctttcccaagcatggcctcctccccccccaagaaaaagcgcaaggtcgccgccgccgattacaaggacgacgacgacaagtcctggaaagacgcgtccggttggtcccgaatgcatgccgcccctcgccgccgcgcggcccagccctccgacgcctcccccgccgcccaagtcgacctccgaaccttgggttactctcagcagcagcaggagaagatcaagcctaaggtccgctccaccgtcgcgcagcatcacgaggccctcgtcggccacggtttcacccatgcccacattgtggccctctcccagcatcccgccgccttgggcacggtggccgtgacgtaccagcacatcatcacggccctccccgaggccacccacgaggatatcgtgggtgtcggtaaacagtggtccggcgcccgcgccttggaggccctcctcaccgatgccggcgaactccgaggtcctcctctccaactcgacaccggccagttggtcaagattgccaagcgcggcggtgtcaccgccatggaggccgtccatgcgtcccgcaacgccttgaccggcgcccccctcaacctgaccccggaccaggtggttgcaatcgcgtcacacgatgggggaaagcaggccctagaaaccgttcagcgactcctgcccgtcctgtgccaggaccacggcctgaccccggaacaggtggttgcaatcgcgtcacacgatgggggaaagcaggccctagaaaccgttcagcgactcctgcccgtcctgtgccaggcccacggcctgaccccagaccaagttgtcgcgattgcaagcaacaacggaggcaaacaagccttagaaacagtccagagattgttgcctgtgctgtgccaagcccacggcctgacccccgcccaggttgtcgctattgctagtaacggcggaggcaaacaggcgctggaaacagttcagcgcctcttgccggtcttgtgtcaggaccacggcctgacccccgaccaggttgtcgctattgctagtaacggcggaggcaaacaggcgctggaaacagttcagcgcctcttgccggtcttgtgtcaggaccacggcctgaccccggaacaggtggttgcaatcgcgtcacacgatgggggaaagcaggccctagaaaccgttcagcgactcctgcccgtcctgtgccaggcccacggcctgaccccggaccaggtggttgcaatcgcgtcacacgatgggggaaagcaggccctagaaaccgttcagcgactcctgcccgtcctgtgccaggcccacggcctgaccccagcccaggttgtggccatcgccagcaacataggtggcaagcaggccctcgaaaccgtccagagactgttaccggttctctgccaggaccacggcctgaccccggaccaggtggttgcaatcgcgtcacacgatgggggaaagcaggccctagaaaccgttcagcgactcctgcccgtcctgtgccaggaccacggcctgaccccagaacaagttgtcgcgattgcaagcaacaacggaggcaaacaagccttagaaacagtccagagattgttgccggtgctgtgccaagcccacggcctgaccccggaccaggtggttgcaatcgcgtcacacgatgggggaaagcaggccctagaaaccgttcagcgactcctgcccgtcctgtgccaggcccacggcctgaccccggcccaggtggttgcaatcgcgtcacacgatgggggaaagcaggccctagaaaccgttcagcgactcctgcccgtcctgtgccaggaccacggcctgaccccggaccaggtggttgcaatcgcgtcacacgatgggggaaagcaggccctagaaaccgttcagcgactcctgcccgtcctgtgccaggaccacggcctgaccccagaacaggttgtggccatcgccagcaacataggtggcaagcaggccctcgaaaccgtccagagactgttaccggttctctgccaggcccacggcctgaccccagaccaagttgtcgcgattgcaagcaacaacggaggcaaacaagccttagaaacagtccagagattgttgcctgtgctgtgccaagcccacggcctgacccccgaacaggtcgtcgccatcgcctctaacggtggtggccgacccgccctcgaatccatcgtggcgcagctctctcgacccgatcccgccttggccgccctcacgaatgaccacctcgtcgccctcgcctgtttgggcggtcgacccgccatggacgcggtcaagaagggcctccctcacgcccctgagctcatccgctcccagctcgtcaagtccgaactcgaggagaagaagtccgagctccgacacaagttgaagtacgtcccccacgagtacatcgagttgatcgagattgcccgcaactccacccaggaccgcatcctcgagatgaaggtcatggagttttttatgaaagtctacggttaccgcggtaagcacctcggtggttcccgcaagcccgatggtgccatctatacggtgggttctcccatcgactacggtgtcatcgtggacaccaaggcgtactccggtggctacaacctccccatcggccaggccgacgagatgcaacgatatgtggaggagaaccagacccgcaacaagcacatcaaccccaacgagtggtggaaggtctacccttcctccgtcaccgagttcaagttcttgtttgtttctggtcatttcaagggtaactacaaggcccaactcacccgactcaaccacatcaccaactgcaacggcgccgtcctctccgtcgaggagctcttgatcggcggcgaaatgatcaaggccggtaccctcaccctcgaggaggtccgccgcaagtttaacaacggcgagatcaacttttgagccgcagcctcttgggtgaagtgtttttaccccccttctccttcacccccgcattcagatgtgcagcgtaaccatacctgctatacataccttgcatcatctagaataactagaaggtcaacgacaatatcttaaaactgagattttgaacgaaagagacttaacaaacagtaggaaataggaagtaatatggaagggatacagctagtagcaaatgattgagtctaagtcctgtcgtttggttcgtgcccgcccctcgtttacatcaagaaatgaaattctcgtcagacagcaggagggagaacattcaccgttaaaagcgtgtagcctttccagagatagagatggaaaagcaagcgacctatcagccgatgaaataatttaaaaagaaaagaaagaaaaggtaacgaggattcaataattgctctgatcctacctagtcgatgataatcttgtctctccttattcttttcggttgtattaatcgggatccatgaccatgattacgccaagctatttaggtgacactataggggaaagcttgcatgcctgcaggtcgactctagaggatctactagtcatatggattggtggagtgagatagcaggagcatcacgcctcacttacggcaaccagcaacagcaacacctgcttgaagcatcaccgcgaacacaggtatgcgcttatggaccttgaacgaatccatgctgcctcaagctcccctccttgcgtgccgtcttgcttgccttaacccttctgcagacgccctagacaagaaataagaggccatccaatagatgattacagatagtggagacccaaaatgctgcacatgcgaccttatttgccattcggggctgagaatcgtgcgcagcgtcgaagccttttttctgcctccctcctctccttccttggatcacttgcttcccattcgcatgtcctgcttgctgcttccctcccccagccaccctcaagtcaaggactttacttccttcttctcacatccaacacaggtgcaactccctccttctttcccaagcatggcctcctccccccccaagaaaaagcgcaaggtcgccgccgccgattacaaggacgacgacgacaagtcctggaaagacgcgtccggttggtcccgaatgcatgccgcccctcgccgccgcgcggcccagccctccgacgcctcccccgccgcccaagtcgacctccgaaccttgggttactctcagcagcagcaggagaagatcaagcctaaggtccgctccaccgtcgcgcagcatcacgaggccctcgtcggccacggtttcacccatgcccacattgtggccctctcccagcatcccgccgccttgggcacggtggccgtgacgtaccagcacatcatcacggccctccccgaggccacccacgaggatatcgtgggtgtcggtaaacagtggtccggcgcccgcgccttggaggccctcctcaccgatgccggcgaactccgaggtcctcctctccaactcgacaccggccagttggtcaagattgccaagcgcggcggtgtcaccgccatggaggccgtccatgcgtcccgcaacgccttgaccggcgcccccctcaacctgaccccggaccaggtggttgcaatcgcgtcacacgatgggggaaagcaggccctagaaaccgttcagcgactcctgcccgtcctgtgccaggaccacggcctgaccccagaacaagttgtcgcgattgcaagcaacaacggaggcaaacaagccttagaaacagtccagagattgttgccggtgctgtgccaagcccacggcctgaccccagaccaggttgtggccatcgccagcaacataggtggcaagcaggccctcgaaaccgtccagagactgttaccggttctctgccaggcccacggcctgacccccgcccaggttgtcgctattgctagtaacggcggaggcaaacaggcgctggaaacagttcagcgcctcttgccggtcttgtgtcaggaccacggcctgaccccagaccaagttgtcgcgattgcaagcaacaacggaggcaaacaagccttagaaacagtccagagattgttgccggtgctgtgccaagaccacggcctgaccccagaacaagttgtcgcgattgcaagcaacaacggaggcaaacaagccttagaaacagtccagagattgttgccggtgctgtgccaagcccacggcctgacccccgaccaggttgtcgctattgctagtaacggcggaggcaaacaggcgctggaaacagttcagcgcctcttgccggtcttgtgtcaggcccacggcctgaccccagcccaagttgtcgcgattgcaagcaacaacggaggcaaacaagccttagaaacagtccagagattgttgccggtgctgtgccaagaccacggcctgaccccggaccaggtggttgcaatcgcgtcacacgatgggggaaagcaggccctagaaaccgttcagcgactcctgcccgtcctgtgccaggaccacggcctgacccccgaacaggttgtcgctattgctagtaacggcggaggcaaacaggcgctggaaacagttcagcgcctcttgccggtcttgtgtcaggcccacggcctgaccccagaccaagttgtcgcgattgcaagcaacaacggaggcaaacaagccttagaaacagtccagagattgttgcctgtgctgtgccaagcccacggcctgaccccggcccaggtggttgcaatcgcgtcacacgatgggggaaagcaggccctagaaaccgttcagcgactcctgcccgtcctgtgccaggaccacggcctgaccccagaccaagttgtcgcgattgcaagcaacaacggaggcaaacaagccttagaaacagtccagagattgttgccggtgctgtgccaagaccacggcctgaccccagaacaggttgtggccatcgccagcaacataggtggcaagcaggccctcgaaaccgtccagagactgttaccggttctctgccaggcccacggcctgaccccagaccaagttgtcgcgattgcaagcaacaacggaggcaaacaagccttagaaacagtccagagattgttgcctgtgctgtgccaagcccacggcctgaccccagcccaggttgtggccatcgccagcaacataggtggcaagcaggccctcgaaaccgtccagagactgttaccggttctctgccaggaccacggcctgacccccgaacaggtcgtcgccatcgcctctaacggtggtggccgacccgccctcgaatccatcgtggcgcagctctctcgacccgatcccgccttggccgccctcacgaatgaccacctcgtcgccctcgcctgtttgggcggtcgacccgccatggacgcggtcaagaagggcctccctcacgcccctgagctcatccgctcccagctcgtcaagtccgaactcgaggagaagaagtccgagctccgacacaagttgaagtacgtcccccacgagtacatcgagttgatcgagattgcccgcaactccacccaggaccgcatcctcgagatgaaggtcatggagttttttatgaaagtctacggttaccgcggtaagcacctcggtggttcccgcaagcccgatggtgccatctatacggtgggttctcccatcgactacggtgtcatcgtggacaccaaggcgtactccggtggctacaacctccccatcggccaggccgacgagatgcaacgatatgtggaggagaaccagacccgcaacaagcacatcaaccccaacgagtggtggaaggtctacccttcctccgtcaccgagttcaagttcttgtttgtttctggtcatttcaagggtaactacaaggcccaactcacccgactcaaccacatcaccaactgcaacggcgccgtcctctccgtcgaggagctcttgatcggcggcgaaatgatcaaggccggtaccctcaccctcgaggaggtccgccgcaagtttaacaacggcgagatcaacttttgagccgcagcctcttgggtgaagtgtttttaccccccttctccttcacccccgcattcagatgtgcagcgtaaccatacctgctatacataccttgcatcatctagaataactagaaggtcaacgacaatatcttaaaactgagattttgaacgaaagagacttaacaaacagtaggaaataggaagtaatatggaagggatacagctagtagcaaatgattgagtctaagtcctgtcgtttggttcgtgcccgcccctcgtttacatcaagaaatgaaattctcgtcagacagcaggagggagaacattcaccgttaaaagcgtgtagcctttccagagatagagatggaaaagcaagcgacctatcagccgatgaaataatttaaaaagaaaagaaagaaaaggtaacgaggattcaataattgctctgatcctacctagtcgatgataatcttgtctctccttattcttttcggttgtattaatcgcccaatctgaataatgttacaaccaattaaccaattctgattagaaaaactcatcgagcatcaaatgaaactgcaatttattcatatcaggattatcaataccatatttttgaaaaagccgtttctgtaatgaaggagaaaactcaccgaggcagttccataggatggcaagatcctggtatcggtctgcgattccgactcgtccaacatcaatacaacctattaatttcccctcgtcaaaaataaggttatcaagtgagaaatcaccatgagtgacgactgaatccggtgagaatggcaaaagtttatgcatttctttccagacttgttcaacaggccagccattacgctcgtcatcaaaatcactcgcatcaaccaaaccgttattcattcgtgattgcgcctgagcaaggcgaaatacgcgatcgctgttaaaaggacaattacaaacaggaatcgaatgcaaccggcgcagggacactgccagcgcatcaacaatattttcacctgaatcaggatattcttctaatacctggaatgctgtttttccggggatcgcagtggtgagtaaccatgcatcatcaggagtacggataaaatgcttgatggtcggaagaggcataaattccgtcagccagtttagtctgaccatctcatctgtaacatcattggcaacgctacctttgccatgtttcagaaacaactctggcgcatcgggcttcccatacaagcgatagattgtcgcacctgattgcccgacattatcgcgagcccatttatacccatataaatcagcatccatgttggaatttaatcgcggcctcgacgtttcccgttgaatatggctcataacaccccttgtattactgtttatgtaagcagacagttttattgttcatgatgatatatttttatcttgtgcaatgtaacatcagagattttgagacacgggccagagctgcgtaccgagctcgaattcacgatgcggtattttctccttacgcatctgtgcggtatttcacaccaagtgccacctgggtccttttcatcacgtgctataaaaataattataatttaaattttttaatataaatatataaattaaaaatagaaagtaaaaaaagaaattaaagaaaaaatagtttttgttttccgaagatgtaaaagactctagggggatcgccaacaaatactaccttttatcttgctcttcctgctctcaggtattaatgccgaattgtttcatcttgtctgtgtagaagaccacacacgaaaatcctgtgattttacattttacttatcgttaatcgaatgtatatctatttaatctgcttttcttgtctaataaatatatatgtaaagtacgctttttgttgaaattttttaaacctttgtttatttttttttcttcattccgtaactcttctaccttctttatttactttctaaaatccaaatacaaaacataaaaataaataaacacagagtaaattcccaaattattccatcattaaaagatacgaggcgcgtgtaagttacaggcaagcgatcccaaaaggccaggaaccgtaaaaaggccgcgttgctggcgtttttccataggctccgcccccctgacgagcatcacaaaaatcgacgctcaagtcagaggtggcgaaacccgacaggactataaagataccaggcgtttccccctggaagctccctcgtgcgctctcctgttccgaccctgccgcttaccggatacctgtccgcctttctcccttcgggaagcgtggcgctttctcatagctcacgctgtaggtatctcagttcggtgtaggtcgttcgctccaagctgggctgtgtgcacgaaccccccgttcagcccgaccgctgcgccttatccggtaactatcgtcttgagtccaacccggtaagacacgacttatcgccactggcagcagccactggtaacaggattagcagagcgaggtatgtaggcggtgctacagagttcttgaagtggtggcctaactacggctacactagaagaacagtatttggtatctgcgctctgctgaagccagttaccttcggaaaaagagttggtagctcttgatccggcaaacaaaccaccgctggtagcggtggtttttttgtttgcaagcagcagattacgcgcagaaaaaaaggatctcaagaagatcctttgatcttttctacggggtctgacgctcagtggaacgaaaactcacgttaagggattttggtcatgagattatcaaaaaggatcttcacctagatccttttaaattaaaaatgaagttttaaatcaatctaaagtatatatgagtaaacttggtctgacagttaccaatgcttaatcagtgaggcacctatctcagcgatctgtctatttcgttcatccatagttgcctgactccccgtcgtgtagataactacgatacgggagggcttaccatctggccccagtgctgcaatgataccgcgagacccacgctcaccggctccagatttatcagcaataaaccagccagccggaagggccgagcgcagaagtggtcctgcaactttatccgcctccatccagtctattaattgttgccgggaagctagagtaagtagttcgccagttaatagtttgcgcaacgttgttgccattgctacaggcatcgtggtgtcacgctcgtcgtttggtatggcttcattcagctccggttcccaacgatcaaggcgagttacatgatcccccatgttgtgcaaaaaagcggttagctccttcggtcctccgatcgttgtcagaagtaagttggccgcagtgttatcactcatggttatggcagcactgcataattctcttactgtcatgccatccgtaagatgcttttctgtgactggtgagtactcaaccaagtcattctgagaatagtgtatgcggcgaccgagttgctcttgcccggcgtcaatacgggataataccgcgccacatagcagaactttaaaagtgctcatcattggaaaacgttcttcggggcgaaaactctcaaggatcttaccgctgttgagatccagttcgatgtaacccactcgtgcacccaactgatcttcagcatcttttactttcaccagcgtttctgggtgagcaaaaacaggaaggcaaaatgccgcaaaaaagggaataagggcgacacggaaatgttgaatactcatactcttcctttttcaatattattgaagcatttatcagggttattgtctcatgagcggatacatatttgaatgtatttagaaaaataaacaaataggggttccgcgcacatttccccgaaaagtgccacctgacgtctaagaaaccattattatcatgacattaacctataaaaataggcgtatcacgaggccctttcgtctggcgcgtttcggtgatgacggtgaaaacctctgacacatgcagctcccgatatcggtcacagcttgtctgtaagcggatgccgggagcagacaagcccgtcagggcgcgtcagcgggtgttggcgggtgtcgggatgaccatgattacgccaagctatttaggtgacactataggggaaagcttgcatgcctgcaggtcgactctagaggatctactagtcatatggattggtggagtgagatagcaggagcatcacgcctcacttacggcaaccagcaacagcaacacctgcttgaagcatcaccgcgaacacaggtatgcgcttatggaccttgaacgaatccatgctgcctcaagctcccctccttgcgtgccgtcttgcttgccttaacccttctgcagacgccctagacaagaaataagaggccatccaatagatgattacagatagtggagacccaaaatgctgcacatgcgaccttatttgccattcggggctgagaatcgtgcgcagcgtcgaagccttttttctgcctccctcctctccttccttggatcacttgcttcccattcgcatgtcctgcttgctgcttccctcccccagccaccctcaagtcaaggactttacttccttcttctcacatccaacacaggtgcaactccctccttctttcccaagcatggacgatgcgttgcgtgcactgcggggtcggtatcccggttgtgagtgggttgttgtggaggatggggcctcgggggctggtgtttatcggcttcggggtggtgggcgggagttgtttgtcaaggtggcagctctgggggccggggtgggcttgttgggtgaggctgagcggctggtgtggttggcggaggtggggattcccgtacctcgtgttgtggagggtggtggggacgagagggtcgcctggttggtcaccgaagcggttccggggcgtccggccagtgcgcggtggccgcgggagcagcggctggacgtggcggtggcgctcgcggggctcgctcgttcgctgcacgcgctggactgggagcggtgtccgttcgatcgcagtctcgcggtgacggtgtagtccgttccacgcccaggcaacaaaactatgccgtctcgcagcaccatcgactgggcttcgtaaatccatcagcactcacactgcctcccacataccatacacgatacacaggcacgcgtccggaggtgccggtgacggtaatttttctccgtgggactgtcggccatcgtaaggaacaaggccggcaaccaaggccaccagggcttattgcgaatcaagcacatccgttccacgcccaggcaacaaaactgtctctaagatggagtggatggaggaggaggcgagcgtagcagcaagcgtgagttatacagccaggcacatgtcgcaatccttcggtctcgggcttaaaatccacgcactaatcacgctgggccatgcaaagagcaatgccgaggcccaccacacaaaacgctgtgtcgcgcgttgcggcctgaagcttcatacttcttagtcgccgccaaaagggctcgagagacgagacccgttggcatgaccgatgttgttcgacgcggtttgcttcgtcacagtcgacgtgattcaggaatctggagcctgcagatcatttttttcagcctgatatcgttcttttccactgagaaccatcagaccaccttttcttccattgtgtgaaggagtaggagttgccgtgctgctttgtgggagacatctgcgatggtgaccagcctcccgtcgtctggtcgacgtgacgagcctcttcactgttcttcgacggagagacgcaagcgagacggctctagaccttttggacacgcattctgtgtgtgaactagtggacagtgataccacgtctgaaagctcaccactgcccatggtgcagctacttgtcacaaagttttgactccgtcggtatcaccattcgcgctcgtgtgcctggttgttccgccacgccggcctgccccggggcggggcaatattctaaaatctcacgcaaaacaccgcacttacccctcacacatattcgtgatagaccaccaccaatctcagcccgcatcaacaatgccgtctcgcagcaccatcgaggtcattaaggctgataagaaccagaacaatctggcgtatggcctaatcgttgtcattcttttggccattgatcccaagtaagtcattctgtcctcaaacatgccttgcttctttcaacacgacgacacggacacttcacactgagacacacgatgtgtgtctgcatgagtatgtaccgccttcatccgttccacgcccaggcaacaaaactatgccgtctcgcagcaccatcgatagattcccgtacctcgtgttgtggagggtggtggggacgagagggtcgcctggttggtcaccgaagcggttccggggcgtccggccagtgcgcggtggccgcgggagcagcggctggacgtggcggtggcgctcgcggggctcgctcgttcgctgcacgcgctggactgggagcggtgtccgttcgatcgcagtctcgcggtgacggtgccgcaggcggcccgtgctgtcgctgaagggagcgtcgacttggaggatctggacgaggagcggaaggggtggtcgggggagcggcttctcgccgagctggagcggactcggcctgcggacgaggatctggcggtttgccacggtgacctgtgcccggacaacgtgctgctcgaccctcgtacctgcgaggtgaccgggctgatcgacgtggggcgggtcggccgtgcggaccggcactccgatctcgcgctggtgctgcgcgagctggcccacgaggaggacccgtggttcgggccggagtgttccgcggcgttcctgcgggagtacgggcgcgggtgggatggggcggtatcggaggaaaagctggcgttttaccggctgttggacgaatttttctgagccgcagcctcttgggtgaagtgtttttaccccccttctccttcacccccgcattcagatgtgcagcgtaaccatacctgctatacataccttgcatcatctagaataactagaaggtcaacgacaatatcttaaaactgagattttgaacgaaagagacttaacaaacagtaggaaataggaagtaatatggaagggatacagctagtagcaaatgattgagtctaagtcctgtcgtttggttcgtgcccgcccctcgtttacatcaagaaatgaaattctcgtcagacagcaggagggagaacattcaccgttaaaagcgtgtagcctttccagagatagagatggaaaagcaagcgacctatcagccgatgaaataatttaaaaagaaaagaaagaaaaggtaacgaggattcaataattgctctgatcctacctagtcgatgataatcttgtctctccttattcttttcggttgtatt

SEQ ID NO: 38 - DNA, 414 bp, synthetic construct
  source 1..414: mol_type = other DNA
ggggaaggaaaaagtgagctcgttcgttcaacgaagttctttgtgcggcggccaaagacagggagagggacgacgggggtaggacgctcggatagttactgagtgaggagggagattacgtgaaacgtgccatcagctccacatgtttttgcacagcaaaagggcgagaggaagtagagttatgcaagtgtaacacacgccataccatacacgttgaacatgaacatcaggtctcttatcttcttgctcactcaccactctgctccccatacactctcttcaccaacgaaaccttgtgcaggacacggtgttgttgtcaaggtcatagcatattaaagaagaccgacggcacaaccgtccgcttaggtggtttctgcgttgttccgtccgccctccgcacaaggagtctggaac

SEQ ID NO: 39 - DNA, 414 bp, synthetic construct
  source 1..414: mol_type = other DNA
atgagcccgcaaggagaggacggcggccccgccgactcgacgacgacgaggacgacgacgtctgaggcgatggccatgccggcaggagcagcagggacagcagccacatctgcatcagacagtcctagcagtcaccaagatgaagggggtggtcctacccaaacggtccaccgcgggccacacccggacattcacgaccagggggacaagacgaaaaagaagaaaaagaagaggaaggatagaaaactccagaatgagagcgaggaccagcagcaacaagacaccgacagccacgcatcaagtcgccccaccactccgatcaacatgacccctccccgctcatcccacgcccgcagccctttcggcgctggctctccatatgaacataccctcacaccttccaacatcgacatt

SEQ ID NO: 40 - DNA, 15541 bp, synthetic construct
  source 1..15541: mol_type = other DNA
ttcctgcgttatcccctgattctgtggataaccgtattaccgcctttgagtgagctgataccgctcgccgcagccgaacgaccgagcgcagcgagtcagtgagcgaggaagcggaagagcgcccaatacgcaaaccgcctctccccgcgcgttggccgattcattaatgcagctgcggccgcatgaccatgattacgccaagctatttaggtgacactataggggaaagcttgcatgcctgcaggtcgactctagaggatctactagtcatatggattggtggagtgagatagcaggagcatcacgcctcacttacggcaaccagcaacagcaacacctgcttgaagcatcaccgcgaacacaggtatgcgcttatggaccttgaacgaatccatgctgcctcaagctcccctccttgcgtgccgtcttgcttgccttaacccttctgcagacgccctagacaagaaataagaggccatccaatagatgattacagatagtggagacccaaaatgctgcacatgcgaccttatttgccattcggggctgagaatcgtgcgcagcgtcgaagccttttttctgcctccctcctctccttccttggatcacttgcttcccattcgcatgtcctgcttgctgcttccctcccccagccaccctcaagtcaaggactttacttccttcttctcacatccaacacaggtgcaactccctccttctttcccaagcatggcctcctccccccccaagaaaaagcgcaaggtcgccgccgccgattacaaggacgacgacgacaagtcctggaaagacgcgtccggttggtcccgaatgcatgccgcccctcgccgccgcgcggcccagccctccgacgcctcccccgccgcccaagtcgacctccgaaccttgggttactctcagcagcagcaggagaagatcaagcctaaggtccgctccaccgtcgcgcagcatcacgaggccctcgtcggccacggtttcacccatgcccacattgtggccctctcccagcatcccgccgccttgggcacggtggccgtgacgtaccagcacatcatcacggccctccccgaggccacccacgaggatatcgtgggtgtcggtaaacagtggtccggcgcccgcgccttggaggccctcctcaccgatgccggcgaactccgaggtcctcctctccaactcgacaccggccagttggtcaagattgccaagcgcggcggtgtcaccgccatggaggccgtccatgcgtcccgcaacgccttgaccggcgcccccctcaacctgaccccggaccaggtggttgcaatcgcgtcacacgatgggggaaagcaggccctagaaaccgttcagcgactcctgcccgtcctgtgccaggaccacggcctgacccccgaacaggttgtcgctattgctagtaacggcggaggcaaacaggcgctggaaacagttcagcgcctcttgccggtcttgtgtcaggcccacggcctgaccccagaccaagttgtcgcgattgcaagcaacaacggaggcaaacaagccttagaaacagtccagagattgttgcctgtgctgtgccaagcccacggcctgaccccagcccaagttgtcgcgattgcaagcaacaacggaggcaaacaagccttagaaacagtccagagattgttgccggtgctgtgccaagaccacggcctgaccccagaccaggttgtggccatcgccagcaacataggtggcaagcaggccctcgaaaccgtccagagactgttaccggttctctgccaggaccacggcctgaccccagaacaggttgtggccatcgccagcaacataggtggcaagcaggccctcgaaaccgtccagagactgttaccggttctctgccaggcccacggcctgaccccggaccaggtggttgcaatcgcgtcacacgatgggggaaagcaggccctagaaaccgttcagcgactcctgcccgtcctgtgccaggcccacggcctgaccccagcccaggttgtggccatcgccagcaacataggtggcaagcaggccctcgaaaccgtccagagactgttaccggttctctgccaggaccacggcctgacccccgaccaggttgtcgctattgctagtaacggcggaggcaaacaggcgctggaaacagttcagcgcctcttgccggtcttgtgtcaggaccacggcctgaccccagaacaagttgtcgcgattgcaagcaacaacggaggcaaacaagccttagaaacagtccagagattgttgccggtgctgtgccaagcccacggcctgaccccagaccaggttgtggccatcgccagcaacataggtggcaagcaggccctcgaaaccgtccagagactgttaccggttctctgccaggcccacggcctgaccccagcccaagttgtcgcgattgcaagcaacaacggaggcaaacaagccttagaaacagtccagagattgttgccggtgctgtgccaagaccacggcctgaccccggaccaggtggttgcaatcgcgtcacacgatgggggaaagcaggccctagaaaccgttcagcgactcctgcccgtcctgtgccaggaccacggcctgaccccggaacaggtggttgcaatcgcgtcacacgatgggggaaagcaggccctagaaaccgttcagcgactcctgcccgtcctgtgccaggcccacggcctgaccccggaccaggtggttgcaatcgcgtcacacgatgggggaaagcaggccctagaaaccgttcagcgactcctgcccgtcctgtgccaggcccacggcctgaccccagcccaagttgtcgcgattgcaagcaacaacggaggcaaacaagccttagaaacagtccagagattgttgccggtgctgtgccaagaccacggcctgacccccgaacaggtcgtcgccatcgcctctaacggtggtggccgacccgccctcgaatccatcgtggcgcagctctctcgacccgatcccgccttggccgccctcacgaatgaccacctcgtcgccctcgcctgtttgggcggtcgacccgccatggacgcggtcaagaagggcctccctcacgcccctgagctcatccgctcccagctcgtcaagtccgaactcgaggagaagaagtccgagctccgacacaagttgaagtacgtcccccacgagtacatcgagttgatcgagattgcccgcaactccacccaggaccgcatcctcgagatgaaggtcatggagttttttatgaaagtctacggttaccgcggtaagcacctcggtggttcccgcaagcccgatggtgccatctatacggtgggttctcccatcgactacggtgtcatcgtggacaccaaggcgtactccggtggctacaacctccccatcggccaggccgacgagatgcaacgatatgtggaggagaaccagacccgcaacaagcacatcaaccccaacgagtggtggaaggtctacccttcctccgtcaccgagttcaagttcttgtttgtttctggtcatttcaagggtaactacaaggcccaactcacccgactcaaccacatcaccaactgcaacggcgccgtcctctccgtcgaggagctcttgatcggcggcgaaatgatcaaggccggtaccctcaccctcgaggaggtccgccgcaagtttaacaacggcgagatcaacttttgagccgcagcctcttgggtgaagtgtttttaccccccttctccttcacccccgcattcagatgtgcagcgtaaccatacctgctatacataccttgcatcatctagaataactagaaggtcaacgacaatatcttaaaactgagattttgaacgaaagagacttaacaaacagtaggaaataggaagtaatatggaagggatacagctagtagcaaatgattgagtctaagtcctgtcgtttggttcgtgcccgcccctcgtttacatcaagaaatgaaattctcgtcagacagcaggagggagaacattcaccgttaaaagcgtgtagcctttccagagatagagatggaaaagcaagcgacctatcagccgatgaaataatttaaaaagaaaagaaagaaaaggtaacgaggattcaataattgctctgatcctacctagtcgatgataatcttgtctctccttattcttttcggttgtattaatcgggatccatgaccatgattacgccaagctatttaggtgacactataggggaaagcttgcatgcctgcaggtcgactctagaggatctactagtcatatggattggtggagtgagatagcaggagcatcacgcctcacttacggcaaccagcaacagcaacacctgcttgaagcatcaccgcgaacacaggtatgcgcttatggaccttgaacgaatccatgctgcctcaagctcccctccttgcgtgccgtcttgcttgccttaacccttctgcagacgccctagacaagaaataagaggccatccaatagatgattacagatagtggagacccaaaatgctgcacatgcgaccttatttgccattcggggctgagaatcgtgcgcagcgtcgaagccttttttctgcctccctcctctccttccttggatcacttgcttcccattcgcatgtcctgcttgctgcttccctcccccagccaccctcaagtcaaggactttacttccttcttctcacatccaacacaggtgcaactccctccttctttcccaagcatggcctcctccccccccaagaaaaagcgcaaggtcgccgccgccgattacaaggacgacgacgacaagtcctggaaagacgcgtccggttggtcccgaatgcatgccgcccctcgccgccgcgcggcccagccctccgacgcctcccccgccgcccaagtcgacctccgaaccttgggttactctcagcagcagcaggagaagatcaagcctaaggtccgctccaccgtcgcgcagcatcacgaggccctcgtcggccacggtttcacccatgcccacattgtggccctctcccagcatcccgccgccttgggcacggtggccgtgacgtaccagcacatcatcacggccctccccgaggccacccacgaggatatcgtgggtgtcggtaaacagtggtccggcgcccgcgccttggaggccctcctcaccgatgccggcgaactccgaggtcctcctctccaactcgacaccggccagttggtcaagattgccaagcgcggcggtgtcaccgccatggaggccgtccatgcgtcccgcaacgccttgaccggcgcccccctcaacctgaccccggaccaggtggttgcaatcgcgtcacacgatgggggaaagcaggccctagaaaccgttcagcgactcctgcccgtcctgtgccaggaccacggcctgaccccagaacaagttgtcgcgattgcaagcaacaacggaggcaaacaagccttagaaacagtccagagattgttgccggtgctgtgccaagcccacggcctgacccccgaccaggttgtcgctattgctagtaacggcggaggcaaacaggcgctggaaacagttcagcgcctcttgccggtcttgtgtcaggcccacggcctgaccccggcccaggtggttgcaatcgcgtcacacgatgggggaaagcaggccctagaaaccgttcagcgactcctgcccgtcctgtgccaggaccacggcctgaccccagaccaagttgtcgcgattgcaagcaacaacggaggcaaacaagccttagaaacagtccagagattgttgccggtgctgtgccaagaccacggcctgaccccagaacaggttgtggccatcgccagcaacataggtggcaagcaggccctcgaaaccgtccagagactgttaccggttctctgccaggcccacggcctgaccccggaccaggtggttgcaatcgcgtcacacgatgggggaaagcaggccctagaaaccgttcagcgactcctgcccgtcctgtgccaggcccacggcctgacccccgcccaggttgtcgctattgctagtaacggcggaggcaaacaggcgctggaaacagttcagcgcctcttgccggtcttgtgtcaggaccacggcctgaccccggaccaggtggttgcaatcgcgtcacacgatgggggaaagcaggccctagaaaccgttcagcgactcctgcccgtcctgtgccaggaccacggcctgaccccagaacaagttgtcgcgattgcaagcaacaacggaggcaaacaagccttagaaacagtccagagattgttgccggtgctgtgccaagcccacggcctgaccccagaccaagttgtcgcgattgcaagcaacaacggaggcaaacaagccttagaaacagtccagagattgttgcctgtgctgtgccaagcccacggcctgaccccggcccaggtggttgcaatcgcgtcacacgatgggggaaagcaggccctagaaaccgttcagcgactcctgcccgtcctgtgccaggaccacggcctgaccccagaccaagttgtcgcgattgcaagcaacaacggaggcaaacaagccttagaaacagtccagagattgttgccggtgctgtgccaagaccacggcctgaccccagaacaagttgtcgcgattgcaagcaacaacggaggcaaacaagccttagaaacagtccagagattgttgccggtgctgtgccaagcccacggcctgaccccagaccaagttgtcgcgattgcaagcaacaacggaggcaaacaagccttagaaacagtccagagattgttgcctgtgctgtgccaagcccacggcctgaccccagcccaagttgtcgcgattgcaagcaacaacggaggcaaacaagccttagaaacagtccagagattgttgccggtgctgtgccaagaccacggcctgacccccgaacaggtcgtcgccatcgcctctaacggtggtggccgacccgccctcgaatccatcgtggcgcagctctctcgacccgatcccgccttggccgccctcacgaatgaccacctcgtcgccctcgcctgtttgggcggtcgacccgccatggacgcggtcaagaagggcctccctcacgcccctgagctcatccgctcccagctcgtcaagtccgaactcgaggagaagaagtccgagctccgacacaagttgaagtacgtcccccacgagtacatcgagttgatcgagattgcccgcaactccacccaggaccgcatcctcgagatgaaggtcatggagttttttatgaaagtctacggttaccgcggtaagcacctcggtggttcccgcaagcccgatggtgccatctatacggtgggttctcccatcgactacggtgtcatcgtggacaccaaggcgtactccggtggctacaacctccccatcggccaggccgacgagatgcaacgatatgtggaggagaaccagacccgcaacaagcacatcaaccccaacgagtggtggaaggtctacccttcctccgtcaccgagttcaagttcttgtttgtttctggtcatttcaagggtaactacaaggcccaactcacccgactcaaccacatcaccaactgcaacggcgccgtcctctccgtcgaggagctcttgatcggcggcgaaatgatcaaggccggtaccctcaccctcgaggaggtccgccgcaagtttaacaacggcgagatcaacttttgagccgcagcctcttgggtgaagtgtttttaccccccttctccttcacccccgcattcagatgtgcagcgtaaccatacctgctatacataccttgcatcatctagaataactagaaggtcaacgacaatatcttaaaactgagattttgaacgaaagagacttaacaaacagtaggaaataggaagtaatatggaagggatacagctagtagcaaatgattgagtctaagtcctgtcgtttggttcgtgcccgcccctcgtttacatcaagaaatgaaattctcgtcagacagcaggagggagaacattcaccgttaaaagcgtgtagcctttccagagatagagatggaaaagcaagcgacctatcagccgatgaaataatttaaaaagaaaagaaagaaaaggtaacgaggattcaataattgctctgatcctacctagtcgatgataatcttgtctctccttattcttttcggttgtattaatcgcccaatctgaataatgttacaaccaattaaccaattctgattagaaaaactcatcgagcatcaaatgaaactgcaatttattcatatcaggattatcaataccatatttttgaaaaagccgtttctgtaatgaaggagaaaactcaccgaggcagttccataggatggcaagatcctggtatcggtctgcgattccgactcgtccaacatcaatacaacctattaatttcccctcgtcaaaaataaggttatcaagtgagaaatcaccatgagtgacgactgaatccggtgagaatggcaaaagtttatgcatttctttccagacttgttcaacaggccagccattacgctcgtcatcaaaatcactcgcatcaaccaaaccgttattcattcgtgattgcgcctgagcaaggcgaaatacgcgatcgctgttaaaaggacaattacaaacaggaatcgaatgcaaccggcgcagggacactgccagcgcatcaacaatattttcacctgaatcaggatattcttctaatacctggaatgctgtttttccggggatcgcagtggtgagtaaccatgcatcatcaggagtacggataaaatgcttgatggtcggaagaggcataaattccgtcagccagtttagtctgaccatctcatctgtaacatcattggcaacgctacctttgccatgtttcagaaacaactctggcgcatcgggcttcccatacaagcgatagattgtcgcacctgattgcccgacattatcgcgagcccatttatacccatataaatcagcatccatgttggaatttaatcgcggcctcgacgtttcccgttgaatatggctcataacaccccttgtattactgtttatgtaagcagacagttttattgttcatgatgatatatttttatcttgtgcaatgtaacatcagagattttgagacacgggccagagctgcgtaccgagctcgaattcacgatgcggtattttctccttacgcatctgtgcggtatttcacaccaagtgccacctgggtccttttcatcacgtgctataaaaataattataatttaaattttttaatataaatatataaattaaaaatagaaagtaaaaaaagaaattaaagaaaaaatagtttttgttttccgaagatgtaaaagactctagggggatcgccaacaaatactaccttttatcttgctcttcctgctctcaggtattaatgccgaattgtttcatcttgtctgtgtagaagaccacacacgaaaatcctgtgattttacattttacttatcgttaatcgaatgtatatctatttaatctgcttttcttgtctaataaatatatatgtaaagtacgctttttgttgaaattttttaaacctttgtttatttttttttcttcattccgtaactcttctaccttctttatttactttctaaaatccaaatacaaaacataaaaataaataaacacagagtaaattcccaaattattccatcattaaaagatacgaggcgcgtgtaagttacaggcaagcgatcccaaaaggccaggaaccgtaaaaaggccgcgttgctggcgtttttccataggctccgcccccctgacgagcatcacaaaaatcgacgctcaagtcagaggtggcgaaacccgacaggactataaagataccaggcgtttccccctggaagctccctcgtgcgctctcctgttccgaccctgccgcttaccggatacctgtccgcctttctcccttcgggaagcgtggcgctttctcatagctcacgctgtaggtatctcagttcggtgtaggtcgttcgctccaagctgggctgtgtgcacgaaccccccgttcagcccgaccgctgcgccttatccggtaactatcgtcttgagtccaacccggtaagacacgacttatcgccactggcagcagccactggtaacaggattagcagagcgaggtatgtaggcggtgctacagagttcttgaagtggtggcctaactacggctacactagaagaacagtatttggtatctgcgctctgctgaagccagttaccttcggaaaaagagttggtagctcttgatccggcaaacaaaccaccgctggtagcggtggtttttttgtttgcaagcagcagattacgcgcagaaaaaaaggatctcaagaagatcctttgatcttttctacggggtctgacgctcagtggaacgaaaactcacgttaagggattttggtcatgagattatcaaaaaggatcttcacctagatccttttaaattaaaaatgaagttttaaatcaatctaaagtatatatgagtaaacttggtctgacagttaccaatgcttaatcagtgaggcacctatctcagcgatctgtctatttcgttcatccatagttgcctgactccccgtcgtgtagataactacgatacgggagggcttaccatctggccccagtgctgcaatgataccgcgagacccacgctcaccggctccagatttatcagcaataaaccagccagccggaagggccgagcgcagaagtggtcctgcaactttatccgcctccatccagtctattaattgttgccgggaagctagagtaagtagttcgccagttaatagtttgcgcaacgttgttgccattgctacaggcatcgtggtgtcacgctcgtcgtttggtatggcttcattcagctccggttcccaacgatcaaggcgagttacatgatcccccatgttgtgcaaaaaagcggttagctccttcggtcctccgatcgttgtcagaagtaagttggccgcagtgttatcactcatggttatggcagcactgcataattctcttactgtcatgccatccgtaagatgcttttctgtgactggtgagtactcaaccaagtcattctgagaatagtgtatgcggcgaccgagttgctcttgcccggcgtcaatacgggataataccgcgccacatagcagaactttaaaagtgctcatcattggaaaacgttcttcggggcgaaaactctcaaggatcttaccgctgttgagatccagttcgatgtaacccactcgtgcacccaactgatcttcagcatcttttactttcaccagcgtttctgggtgagcaaaaacaggaaggcaaaatgccgcaaaaaagggaataagggcgacacggaaatgttgaatactcatactcttcctttttcaatattattgaagcatttatcagggttattgtctcatgagcggatacatatttgaatgtatttagaaaaataaacaaataggggttccgcgcacatttccccgaaaagtgccacctgacgtctaagaaaccattattatcatgacattaacctataaaaataggcgtatcacgaggccctttcgtctggcgcgtttcggtgatgacggtgaaaacctctgacacatgcagctcccgatatcggtcacagcttgtctgtaagcggatgccgggagcagacaagcccgtcagggcgcgtcagcgggtgttggcgggtgtcgggatgaccatgattacgccaagctatttaggtgacactataggggaaagcttgcatgcctgcaggtcgactctagaggatctactagtcatatggattggtggagtgagatagcaggagcatcacgcctcacttacggcaaccagcaacagcaacacctgcttgaagcatcaccgcgaacacaggtatgcgcttatggaccttgaacgaatccatgctgcctcaagctcccctccttgcgtgccgtcttgcttgccttaacccttctgcagacgccctagacaagaaataagaggccatccaatagatgattacagatagtggagacccaaaatgctgcacatgcgaccttatttgccattcggggctgagaatcgtgcgcagcgtcgaagccttttttctgcctccctcctctccttccttggatcacttgcttcccattcgcatgtcctgcttgctgcttccctcccccagccaccctcaagtcaaggactttacttccttcttctcacatccaacacaggtgcaactccctccttctttcccaagcatggacgatgcgttgcgtgcactgcggggtcggtatcccggttgtgagtgggttgttgtggaggatggggcctcgggggctggtgtttatcggcttcggggtggtgggcgggagttgtttgtcaaggtggcagctctgggggccggggtgggcttgttgggtgaggctgagcggctggtgtggttggcggaggtggggattcccgtacctcgtgttgtggagggtggtggggacgagagggtcgcctggttggtcaccgaagcggttccggggcgtccggccagtgcgcggtggccgcgggagcagcggctggacgtggcggtggcgctcgcggggctcgctcgttcgctgcacgcgctggactgggagcggtgtccgttcgatcgcagtctcgcggtgacggtgtagtctggaacatgagcccgcaaggagaggacggcggccccgccgactcgacgaggggaaggaaaaagtgagctcgttcgttcaacgaagttctttgtgcggcggccaaagacagggagagggacgacgggggtaggacgctcggatagttactgagtgaggagggagattacgtgaaacgtgccatcagctccacatgtttttgcacagcaaaagggcgagaggaagtagagttatgcaagtgtaacacacgccataccatacacgttgaacatgaacatcaggtctcttatcttcttgctcactcaccactctgctccccatacactctcttcaccaacgaaaccttgtgcaggacacggtgttgttgtcaaggtcatagcatattaaagaagaccgacggcacaaccgtccgcttaggtggtttctgcgttgttccgtccgccctccgcacaaggagtctggaacgtctctaagatggagtggatggaggaggaggcgagcgtagcagcaagcgtgagttatacagccaggcacatgtcgcaatccttcggtctcgggcttaaaatccacgcactaatcacgctgggccatgcaaagagcaatgccgaggcccaccacacaaaacgctgtgtcgcgcgttgcggcctgaagcttcatacttcttagtcgccgccaaaagggctcgagagacgagacccgttggcatgaccgatgttgttcgacgcggtttgcttcgtcacagtcgacgtgattcaggaatctggagcctgcagatcatttttttcagcctgatatcgttcttttccactgagaaccatcagaccaccttttcttccattgtgtgaaggagtaggagttgccgtgctgctttgtgggagacatctgcgatggtgaccagcctcccgtcgtctggtcgacgtgacgagcctcttcactgttcttcgacggagagacgcaagcgagacggctctagaccttttggacacgcattctgtgtgtgaactagtggacagtgataccacgtctgaaagctcaccactgcccatggtgcagctacttgtcacaaagttttgactccgtcggtatcaccattcgcgctcgtgtgcctggttgttccgccacgccggcctgccccggggcggggcaatattctaaaatctcacgcaaaacaccgcacttacccctcacacatattcgtgatagaccaccaccaatctcagcccgcatcaacaatgagcccgcaaggagaggacggcggccccgccgactcgacgacgacgaggacgacgacgtctgaggcgatggccatgccggcaggagcagcagggacagcagccacatctgcatcagacagtcctagcagtcaccaagatgaagggggtggtcctacccaaacggtccaccgcgggccacacccggacattcacgaccagggggacaagacgaaaaagaagaaaaagaagaggaaggatagaaaactccagaatgagagcgaggaccagcagcaacaagacaccgacagccacgcatcaagtcgccccaccactccgatcaacatgacccctccccgctcatcccacgcccgcagccctttcggcgctggctctccatatgaacataccctcacaccttccaacatcgacatttctggaacatgagcccgcaaggagaggacggcggccccgccgactcgacgatagattcccgtacctcgtgttgtggagggtggtggggacgagagggtcgcctggttggtcaccgaagcggttccggggcgtccggccagtgcgcggtggccgcgggagcagcggctggacgtggcggtggcgctcgcggggctcgctcgttcgctgcacgcgctggactgggagcggtgtccgttcgatcgcagtctcgcggtgacggtgccgcaggcggcccgtgctgtcgctgaagggagcgtcgacttggaggatctggacgaggagcggaaggggtggtcgggggagcggcttctcgccgagctggagcggactcggcctgcggacgaggatctggcggtttgccacggtgacctgtgcccggacaacgtgctgctcgaccctcgtacctgcgaggtgaccgggctgatcgacgtggggcgggtcggccgtgcggaccggcactccgatctcgcgctggtgctgcgcgagctggcccacgaggaggacccgtggttcgggccggagtgttccgcggcgttcctgcgggagtacgggcgcgggtgggatggggcggtatcggaggaaaagctggcgttttaccggctgttggacgaatttttctgagccgcagcctcttgggtgaagtgtttttaccccccttctccttcacccccgcattcagatgtgcagcgtaaccatacctgctatacataccttgcatcatctagaataactagaaggtcaacgacaatatcttaaaactgagattttgaacgaaagagacttaacaaacagtaggaaataggaagtaatatggaagggatacagctagtagcaaatgattgagtctaagtcctgtcgtttggttcgtgcccgcccctcgtttacatcaagaaatgaaattctcgtcagacagcaggagggagaacattcaccgttaaaagcgtgtagcctttccagagatagagatggaaaagcaagcgacctatcagccgatgaaataatttaaaaagaaaagaaagaaaaggtaacgaggattcaataattgctctgatcctacctagtcgatgataatcttgtctctccttattcttttcggttgtatt

SEQ ID NO: 41 - DNA, 204 bp, synthetic construct
  source 1..204: mol_type = other DNA
gtgatgcggttttggcagtacatcaatgggcgtggatagcggtttgactcacggggatttccaagtctccaccccattgacgtcaatgggagtttgttttggcaccaaaatcaacgggactttccaaaatgtcgtaacaactccgccccattgacgcaaatgggcggtaggcgtgtacggtgggaggtctatataagcagagct

SEQ ID NO: 42 - DNA, 225 bp, synthetic construct
  source 1..225: mol_type = other DNA
ctgtgccttctagttgccagccatctgttgtttgcccctcccccgtgccttccttgaccctggaaggtgccactcccactgtcctttcctaataaaatgaggaaattgcatcgcattgtctgagtaggtgtcattctattctggggggtggggtggggcaggacagcaagggggaggattgggaagacaatagcaggcatgctggggatgcggtgggctctatgg

SEQ ID NO: 43 - DNA, 417 bp, synthetic construct
  source 1..417: mol_type = other DNA
atgaccgagtacaagcccacggtgcgcctcgccacccgcgacgacgtccccagggccgtacgcaccctcgccgccgcgttcgccgactaccccgccacgcgccacaccgtcgatccggaccgccacatcgagcgggtcaccgagctgcaagaactcttcctcacgcgcgtcgggctcgacatcggcaaggtgtgggtcgcggacgacggcgccgcggtggcggtctggaccacgccggagagcgtcgaagcgggggcggtgttcgccgagatcggcccgcgcatggccgagttgagcggttcccggctggccgcgcagcaacagatggaaggcctcctggcgccgcaccggcccaaggagcccgcgtggttcctggccaccgtcggcgtctcgcccgaccaccagggcaagggtctg

SEQ ID NO: 44 - DNA, 242 bp, synthetic construct
  source 1..242: mol_type = other DNA
gagcccgcgtggttcctggccaccgtcggcgtctcgcccgaccaccagggcaagggtctgggcagcgccgtcgtgctccccggagtggaggcggccgagcgcgccggggtgcccgccttcctggagacctccgcgccccgcaacctccccttctacgagcggctcggcttcaccgtcaccgccgacgtcgaggtgcccgaaggaccgcgcacctggtgcatgacccgcaagcccggtgcctg

SEQ ID NO: 45 - DNA, 23 bp, synthetic construct
  source 1..23: mol_type = other DNA
gtgcttcgatatcgatcgtttgg

SEQ ID NO: 46 - DNA, 23 bp, synthetic construct
  source 1..23: mol_type = other DNA
ccaaacgatcgatatcgaagcac

SEQ ID NO: 47 - DNA, 66 bp, synthetic construct
  source 1..66: mol_type = other DNA
gactataaggaccacgacggagactacaaggatcatgatattgattacaaagacgatgacgataag

SEQ ID NO: 48 - DNA, 40 bp, synthetic construct
  source 1..40: mol_type = other DNA
atctgctgaaactgaaattcaattttaagacctccctgtg

SEQ ID NO: 49 - DNA, 40 bp, synthetic construct
  source 1..40: mol_type = other DNA
gtaattgggagaggtagccgagtcacacccggtggctctg

SEQ ID NO: 50 - DNA, 4766 bp, synthetic construct
  source 1..4766: mol_type = other DNA
attaaaaatgaagttttaaatcaatctaaagtatatatgagtaaacttggtctgacagttaccaatgcttaatcagtgaggcacctatctcagcgatctgtctatttcgttcatccatagttgcctgactccccgtcgtgtagataactacgatacgggagggcttaccatctggccccagtgctgcaatgataccgcgagacccacgctcaccggctccagatttatcagcaataaaccagccagccggaagggccgagcgcagaagtggtcctgcaactttatccgcctccatccagtctattaattgttgccgggaagctagagtaagtagttcgccagttaatagtttgcgcaacgttgttgccattgctacaggcatcgtggtgtcacgctcgtcgtttggtatggcttcattcagctccggttcccaacgatcaaggcgagttacatgatcccccatgttgtgcaaaaaagcggttagctccttcggtcctccgatcgttgtcagaagtaagttggccgcagtgttatcactcatggttatggcagcactgcataattctcttactgtcatgccatccgtaagatgcttttctgtgactggtgagtactcaaccaagtcattctgagaatagtgtatgcggcgaccgagttgctcttgcccggcgtcaatacgggataataccgcgccacatagcagaactttaaaagtgctcatcattggaaaacgttcttcggggcgaaaactctcaaggatcttaccgctgttgagatccagttcgatgtaacccactcgtgcacccaactgatcttcagcatcttttactttcaccagcgtttctgggtgagcaaaaacaggaaggcaaaatgccgcaaaaaagggaataagggcgacacggaaatgttgaatactcatactcttcctttttcaatattattgaagcatttatcagggttattgtctcatgagcggatacatatttgaatgtatttagaaaaataaacaaataggggttccgcgcacatttccccgaaaagtgccacctgacgcgccctgtagcggcgcattaagcgcggcgggtgtggtggttacgcgcagcgtgaccgctacacttgccagcgccctagcgcccgctcctttcgctttcttcccttcctttctcgccacgttcgccggctttccccgtcaagctctaaatcgggggctccctttagggttccgatttagtgctttacggcacctcgaccccaaaaaacttgattagggtgatggttcacgtagtgggccatcgccctgatagacggtttttcgccctttgacgttggagtccacgttctttaatagtggactcttgttccaaactggaacaacactcaaccctatctcggtctattcttttgatttataagggattttgccgatttcggcctattggttaaaaaatgagctgatttaacaaaaatttaacgcgaattttaacaaaatattaacgcttacaatttccattcgccattcaggctgcgcaactgttgggaagggcgatcggtgcgggcctcttcgctattacgccagctggcgaaagggggatgtgctgcaaggcgattaagttgggtaacgccagggttttcccagtcacgacgttgtaaaacgacggccagtgagcgcgcgtaatacgactcactatagggcgaattgggtaccgggccccccctcgaggtcgacggtatcgataagcttgatatcgaattgcattcattttatgtttcaggttcagggggaggtgtgggaggttttttaaagcaagtaaaacctctacaaatgtggtacgcgttgacattgattattgactagttattaatagtaatcaattacggggtcattagttcatagcccatatatggagttccgcgttacataacttacggtaaatggcccgcctggctgaccgcccaacgacccccgcccattgacgtcaataatgacgtatgttcccatagtaacgccaatagggactttccattgacgtcaatgggtggagtatttacggtaaactgcccacttggcagtacatcaagtgtatcatatgccaagtacgccccctattgacgtcaatgacggtaaatggcccgcctggcattatgcccagtacatgaccttatgggactttcctacttggcagtacatctacgtattagtcatcgctattaccatggtgatgcggttttggcagtacatcaatgggcgtggatagcggtttgactcacggggatttccaagtctccaccccattgacgtcaatgggagtttgttttggcaccaaaatcaacgggactttccaaaatgtcgtaacaactccgccccattgacgcaaatgggcggtaggcgtgtacggtgggaggtctatataagcagagctctctggctaactagagaacccactgcgccaccatgaccgagtacaagcccacggtgcgcctcgccacccgcgacgacgtccccagggccgtacgcaccctcgccgccgcgttcgccgactaccccgccacgcgccacaccgtcgatccggaccgccacatcgagcgggtcaccgagctgcaagaactcttcctcacgcgcgtcgggctcgacatcggcaaggtgtgggtcgcggacgacggcgccgcggtggcggtctggaccacgccggagagcgtcgaagcgggggcggtgttcgccgagatcggcccgcgcatggccgagttgagcggttcccggctggccgcgcagcaacagatggaaggcctcctggcgccgcaccggcccaaggagcccgcgtggttcctggccaccgtcggcgtctcgcccgaccaccagggcaagggtctgtaggtgcttcgatatcgatcgtttggatctgctgaaactgaaattcaattttaagacctccctgtggggatccgactataaggaccacgacggagactacaaggatcatgatattgattacaaagacgatgacgataagtaagtaattgggagaggtagccgagtcacacccggtggctctgccaaacgatcgatatcgaagcactaagagcccgcgtggttcctggccaccgtcggcgtctcgcccgaccaccagggcaagggtctgggcagcgccgtcgtgctccccggagtggaggcggccgagcgcgccggggtgcccgccttcctggagacctccgcgccccgcaacctccccttctacgagcggctcggcttcaccgtcaccgccgacgtcgaggtgcccgaaggaccgcgcacctggtgcatgacccgcaagcccggtgcctgactcgagtctagagggcccgtttaaacccgctgatcagcctcgactgtgccttctagttgccagccatctgttgtttgcccctcccccgtgccttccttgaccctggaaggtgccactcccactgtcctttcctaataaaatgaggaaattgcatcgcattgtctgagtaggtgtcattctattctggggggtggggtggggcaggacagcaagggggaggattgggaagacaatagcaggcatgctggggatgcggtgggctctatgggcggccgccaccgcggtggagctccagcttttgttccctttagtgagggttaattgcgcgcttggcgtaatcatggtcatagctgtttcctgtgtgaaattgttatccgctcacaattccacacaacatacgagccggaagcataaagtgtaaagcctggggtgcctaatgagtgagctaactcacattaattgcgttgcgctcactgcccgctttccagtcgggaaacctgtcgtgccagctgcattaatgaatcggccaacgcgcggggagaggcggtttgcgtattgggcgctcttccgcttcctcgctcactgactcgctgcgctcggtcgttcggctgcggcgagcggtatcagctcactcaaaggcggtaatacggttatccacagaatcaggggataacgcaggaaagaacatgtgagcaaaaggccagcaaaaggccaggaaccgtaaaaaggccgcgttgctggcgtttttccataggctccgcccccctgacgagcatcacaaaaatcgacgctcaagtcagaggtggcgaaacccgacaggactataaagataccaggcgtttccccctggaagctccctcgtgcgctctcctgttccgaccctgccgcttaccggatacctgtccgcctttctcccttcgggaagcgtggcgctttctcatagctcacgctgtaggtatctcagttcggtgtaggtcgttcgctccaagctgggctgtgtgcacgaaccccccgttcagcccgaccgctgcgccttatccggtaactatcgtcttgagtccaacccggtaagacacgacttatcgccactggcagcagccactggtaacaggattagcagagcgaggtatgtaggcggtgctacagagttcttgaagtggtggcctaactacggctacactagaaggacagtatttggtatctgcgctctgctgaagccagttaccttcggaaaaagagttggtagctcttgatccggcaaacaaaccaccgctggtagcggtggtttttttgtttgcaagcagcagattacgcgcagaaaaaaaggatctcaagaagatcctttgatcttttctacggggtctgacgctcagtggaacgaaaactcacgttaagggattttggtcatgagattatcaaaaaggatcttcacctagatccttttaa

SEQ ID NO: 51 - DNA, 417 bp, synthetic construct; identical to SEQ ID NO: 43
  source 1..417: mol_type = other DNA

SEQ ID NO: 52 - DNA, 375 bp, synthetic construct
  source 1..375: mol_type = other DNA
tggaccacgccggagagcgtcgaagcgggggcggtgttcgccgagatcggcccgcgcatggccgagttgagcggttcccggctggccgcgcagcaacagatggaaggcctcctggcgccgcaccggcccaaggagcccgcgtggttcctggccaccgtcggcgtctcgcccgaccaccagggcaagggtctgggcagcgccgtcgtgctccccggagtggaggcggccgagcgcgccggggtgcccgccttcctggagacctccgcgccccgcaacctccccttctacgagcggctcggcttcaccgtcaccgccgacgtcgaggtgcccgaaggaccgcgcacctggtgcatgacccgcaagcccggtgcctga

SEQ ID NO: 53 - DNA, 4899 bp, synthetic construct
  source 1..4899: mol_type = other DNA
attaaaaatgaagttttaaatcaatctaaagtatatatgagtaaacttggtctgacagttaccaatgcttaatcagtgaggcacctatctcagcgatctgtctatttcgttcatccatagttgcctgactccccgtcgtgtagataactacgatacgggagggcttaccatctggccccagtgctgcaatgataccgcgagacccacgctcaccggctccagatttatcagcaataaaccagccagccggaagggccgagcgcagaagtggtcctgcaactttatccgcctccatccagtctattaattgttgccgggaagctagagtaagtagttcgccagttaatagtttgcgcaacgttgttgccattgctacaggcatcgtggtgtcacgctcgtcgtttggtatggcttcattcagctccggttcccaacgatcaaggcgagttacatgatcccccatgttgtgcaaaaaagcggttagctccttcggtcctccgatcgttgtcagaagtaagttggccgcagtgttatcactcatggttatggcagcactgcataattctcttactgtcatgccatccgtaagatgcttttctgtgactggtgagtactcaaccaagtcattctgagaatagtgtatgcggcgaccgagttgctcttgcccggcgtcaatacgggataataccgcgccacatagcagaactttaaaagtgctcatcattggaaaacgttcttcggggcgaaaactctcaaggatcttaccgctgttgagatccagttcgatgtaacccactcgtgcacccaactgatcttcagcatcttttactttcaccagcgtttctgggtgagcaaaaacaggaaggcaaaatgccgcaaaaaagggaataagggcgacacggaaatgttgaatactcatactcttcctttttcaatattattgaagcatttatcagggttattgtctcatgagcggatacatatttgaatgtatttagaaaaataaacaaataggggttccgcgcacatttccccgaaaagtgccacctgacgcgccctgtagcggcgcattaagcgcggcgggtgtggtggttacgcgcagcgtgaccgctacacttgccagcgccctagcgcccgctcctttcgctttcttcccttcctttctcgccacgttcgccggctttccccgtcaagctctaaatcgggggctccctttagggttccgatttagtgctttacggcacctcgaccccaaaaaacttgattagggtgatggttcacgtagtgggccatcgccctgatagacggtttttcgccctttgacgttggagtccacgttctttaatagtggactcttgttccaaactggaacaacactcaaccctatctcggtctattcttttgatttataagggattttgccgatttcggcctattggttaaaaaatgagctgatttaacaaaaatttaacgcgaattttaacaaaatattaacgcttacaatttccattcgccattcaggctgcgcaactgttgggaagggcgatcggtgcgggcctcttcgctattacgccagctggcgaaagggggatgtgctgcaaggcgattaagttgggtaacgccagggttttcccagtcacgacgttgtaaaacgacggccagtgagcgcgcgtaatacgactcactatagggcgaattgggtaccgggccccccctcgaggtcgacggtatcgataagcttgatatcgaattgcattcattttatgtttcaggttcagggggaggtgtgggaggttttttaaagcaagtaaaacctctacaaatgtggtacgcgttgacattgattattgactagttattaatagtaatcaattacggggtcattagttcatagcccatatatggagttccgcgttacataacttacggtaaatggcccgcctggctgaccgcccaacgacccccgcccattgacgtcaataatgacgtatgttcccatagtaacgccaatagggactttccattgacgtcaatgggtggagtatttacggtaaactgcccacttggcagtacatcaagtgtatcatatgccaagtacgccccctattgacgtcaatgacggtaaatggcccgcctggcattatgcccagtacatgaccttatgggactttcctacttggcagtacatctacgtattagtcatcgctattaccatggtgatgcggttttggcagtacatcaatgggcgtggatagcggtttgactcacggggatttccaagtctccaccccattgacgtcaatgggagtttgttttggcaccaaaatcaacgggactttccaaaatgtcgtaacaactccgccccattgacgcaaatgggcggtaggcgtgtacggtgggaggtctatataagcagagctctctggctaactagagaacccactgcgccaccatgaccgagtacaagcccacggtgcgcctcgccacccgcgacgacgtccccagggccgtacgcaccctcgccgccgcgttcgccgactaccccgccacgcgccacaccgtcgatccggaccgccacatcgagcgggtcaccgagctgcaagaactcttcctcacgcgcgtcgggctcgacatcggcaaggtgtgggtcgcggacgacggcgccgcggtggcggtctggaccacgccggagagcgtcgaagcgggggcggtgttcgccgagatcggcccgcgcatggccgagttgagcggttcccggctggccgcgcagcaacagatggaaggcctcctggcgccgcaccggcccaaggagcccgcgtggttcctggccaccgtcggcgtctcgcccgaccaccagggcaagggtctgtaggtgcttcgatatcgatcgtttggatctgctgaaactgaaattcaattttaagacctccctgtggggatccgactataaggaccacgacggagactacaaggatcatgatattgattacaaagacgatgacgataagtaagtaattgggagaggtagccgagtcacacccggtggctctgccaaacgatcgatatcgaagcactaatggaccacgccggagagcgtcgaagcgggggcggtgttcgccgagatcggcccgcgcatggccgagttgagcggttcccggctggccgcgcagcaacagatggaaggcctcctggcgccgcaccggcccaaggagcccgcgtggttcctggccaccgtcggcgtctcgcccgaccaccagggcaagggtctgggcagcgccgtcgtgctccccggagtggaggcggccgagcgcgccggggtgcccgccttcctggagacctccgcgccccgcaacctccccttctacgagcggctcggcttcaccgtcaccgccgacgtcgaggtgcccgaaggaccgcgcacctggtgcatgacccgcaagcccggtgcctgaactcgagtctagagggcccgtttaaacccgctgatcagcctcgactgtgccttctagttgccagccatctgttgtttgcccctcccccgtgccttccttgaccctggaaggtgccactcccactgtcctttcctaataaaatgaggaaattgcatcgcattgtctgagtaggtgtcattctattctggggggtggggtggggcaggacagcaagggggaggattgggaagacaatagcaggcatgctggggatgcggtgggctctatgggcggccgccaccgcggtggagctccagcttttgttccctttagtgagggttaattgcgcgcttggcgtaatcatggtcatagctgtttcctgtgtgaaattgttatccgctcacaattccacacaacatacgagccggaagcataaagtgtaaagcctggggtgcctaatgagtgagctaactcacattaattgcgttgcgctcactgcccgctttccagtcgggaaacctgtcgtgccagctgcattaatgaatcggccaacgcgcggggagaggcggtttgcgtattgggcgctcttccgcttcctcgctcactgactcgctgcgctcggtcgttcggctgcggcgagcggtatcagctcactcaaaggcggtaatacggttatccacagaatcaggggataacgcaggaaagaacatgtgagcaaaaggccagcaaaaggccaggaaccgtaaaaaggccgcgttgctggcgtttttccataggctccgcccccctgacgagcatcacaaaaatcgacgctcaagtcagaggtggcgaaacccgacaggactataaagataccaggcgtttccccctggaagctccctcgtgcgctctcctgttccgaccctgccgcttaccggatacctgtccgcctttctcccttcgggaagcgtggcgctttctcatagctcacgctgtaggtatctcagttcggtgtaggtcgttcgctccaagctgggctgtgtgcacgaaccccccgttcagcccgaccgctgcgccttatccggtaactatcgtcttgagtccaacccggtaagacacgacttatcgccactggcagcagccactggtaacaggattagcagagcgaggtatgtaggcggtgctacagagttcttgaagtggtggcctaactacggctacactagaaggacagtatttggtatctgcgctctgctgaagccagttaccttcggaaaaagagttggtagctcttgatccggcaaacaaaccaccgctggtagcggtggtttttttgtttgcaagcagcagattacgcgcagaaaaaaaggatctcaagaagatcctttgatcttttctacggggtctgacgctcagtggaacgaaaactcacgttaagggattttggtcatgagattatcaaaaaggatcttcacctagatccttttaa

SEQ ID NO: 54 - DNA, 40 bp, synthetic construct
  source 1..40: mol_type = other DNA
gtggcaaaagctgataagctggctgaagagcattcatcgt

SEQ ID NO: 55 - DNA, 40 bp, synthetic construct
  source 1..40: mol_type = other DNA
gaggggtctttgtcctctgtactgtctctctccttgcccc

SEQ ID NO: 56 - DNA, 4767 bp, synthetic construct
  source 1..4767: mol_type = other DNA
attaaaaatgaagttttaaatcaatctaaagtatatatgagtaaacttggtctgacagttaccaatgcttaatcagtgaggcacctatctcagcgatctgtctatttcgttcatccatagttgcctgactccccgtcgtgtagataactacgatacgggagggcttaccatctggccccagtgctgcaatgataccgcgagacccacgctcaccggctccagatttatcagcaataaaccagccagccggaagggccgagcgcagaagtggtcctgcaactttatccgcctccatccagtctattaattgttgccgggaagctagagtaagtagttcgccagttaatagtttgcgcaacgttgttgccattgctacaggcatcgtggtgtcacgctcgtcgtttggtatggcttcattcagctccggttcccaacgatcaaggcgagttacatgatcccccatgttgtgcaaaaaagcggttagctccttcggtcctccgatcgttgtcagaagtaagttggccgcagtgttatcactcatggttatggcagcactgcataattctcttactgtcatgccatccgtaagatgcttttctgtgactggtgagtactcaaccaagtcattctgagaatagtgtatgcggcgaccgagttgctcttgcccggcgtcaatacgggataataccgcgccacatagcagaactttaaaagtgctcatcattggaaaacgttcttcggggcgaaaactctcaaggatcttaccgctgttgagatccagttcgatgtaacccactcgtgcacccaactgatcttcagcatcttttactttcaccagcgtttctgggtgagcaaaaacaggaaggcaaaatgccgcaaaaaagggaataagggcgacacggaaatgttgaatactcatactcttcctttttcaatattattgaagcatttatcagggttattgtctcatgagcggatacatatttgaatgtatttagaaaaataaacaaataggggttccgcgcacatttccccgaaaagtgccacctgacgcgccctgtagcggcgcattaagcgcggcgggtgtggtggttacgcgcagcgtgaccgctacacttgccagcgccctagcgcccgctcctttcgctttcttcccttcctttctcgccacgttcgccggctttccccgtcaagctctaaatcgggggctccctttagggttccgatttagtgctttacggcacctcgaccccaaaaaacttgattagggtgatggttcacgtagtgggccatcgccctgatagacggtttttcgccctttgacgttggagtccacgttctttaatagtggactcttgttccaaactggaacaacactcaaccctatctcggtctattcttttgatttataagggattttgccgatttcggcctattggttaaaaaatgagctgatttaacaaaaatttaacgcgaattttaacaaaatattaacgcttacaatttccattcgccattcaggctgcgcaactgttgggaagggcgatcggtgcgggcctcttcgctattacgccagctggcgaaagggggatgtgctgcaaggcgattaagttgggtaacgccagggttttcccagtcacgacgttgtaaaacgacggccagtgagcgcgcgtaatacgactcactatagggcgaattgggtaccgggccccccctcgaggtcgacggtatcgataagcttgatatcgaattgcattcattttatgtttcaggttcagggggaggtgtgggaggttttttaaagcaagtaaaacctctacaaatgtggtacgcgttgacattgattattgactagttattaatagtaatcaattacggggtcattagttcatagcccatatatggagttccgcgttacataacttacggtaaatggcccgcctggctgaccgcccaacgacccccgcccattgacgtcaataatgacgtatgttcccatagtaacgccaatagggactttccattgacgtcaatgggtggagtatttacggtaaactgcccacttggcagtacatcaagtgtatcatatgccaagtacgccccctattgacgtcaatgacggtaaatggcccgcctggcattatgcccagtacatgaccttatgggactttcctacttggcagtacatctacgtattagtcatcgctattaccatggtgatgcggttttggcagtacatcaatgggcgtggatagcggtttgactcacggggatttccaagtctccaccccattgacgtcaatgggagtttgttttggcaccaaaatcaacgggactttccaaaatgtcgtaacaactccgccccattgacgcaaatgggcggtaggcgtgtacggtgggaggtctatataagcagagctctctggctaactagagaacccactgcgccaccatgaccgagtacaagcccacggtgcgcctcgccacccgcgacgacgtccccagggccgtacgcaccctcgccgccgcgttcgccgactaccccgccacgcgccacaccgtcgatccggaccgccacatcgagcgggtcaccgagctgcaagaactcttcctcacgcgcgtcgggctcgacatcggcaaggtgtgggtcgcggacgacggcgccgcggtggcggtctggaccacgccggagagcgtcgaagcgggggcggtgttcgccgagatcggcccgcgcatggccgagttgagcggttcccggctggccgcgcagcaacagatggaaggcctcctggcgccgcaccggcccaaggagcccgcgtggttcctggccaccgtcggcgtctcgcccgaccaccagggcaagggtctgtaggtgcttcgatatcgatcgtttgggtggcaaaagctgataagctggctgaagagcattcatcgtggggatccgactataaggaccacgacggagactacaaggatcatgatattgattacaaagacgatgacgataagtaagaggggtctttgtcctctgtactgtctctctccttgccccccaaacgatcgatatcgaagcactaagagcccgcgtggttcctggccaccgtcggcgtctcgcccgaccaccagggcaagggtctgggcagcgccgtcgtgctccccggagtggaggcggccgagcgcgccggggtgcccgccttcctggagacctccgcgccccgcaacctccccttctacgagcggctcggcttcaccgtcaccgccgacgtcgaggtgcccgaaggaccgcgcacctggtgcatgacccgcaagcccggtgcctgactcgagtctagagggcccgtttaaacccgctgatcagcctcgactgtgccttctagttgccagccatctgttgtttgcccctcccccgtgccttccttgaccctggaaggtgccactcccactgtcctttcctaataaaatgaggaaattgcatcgcattgtctgagtaggtgtcattctattctggggggtggggtggggcaggacagcaagggggaggattgggaagacaatagcaggcatgctggggatgcggtgggctctatgggcggccgccaccgcggtggagctccagcttttgttccctttagtgagggttaattgcgcgcttggcgtaatcatggtcatagctgtttcctgtgtgaaattgttatccgctcacaattccacacaacatacgagccggaagcataaagtgtaaagcctggggtgcctaatgagtgagctaactcacattaattgcgttgcgctcactgcccgctttccagtcgggaaacctgtcgtgccagctgcattaatgaatcggccaacgcgcggggagaggcggtttgcgtattgggcgctcttccgcttcctcgctcactgactcgctgcgctcggtcgttcggctgcggcgagcggtatcagctcactcaaaggcggtaatacggttatccacagaatcaggggataacgcaggaaagaacatgtgagcaaaaggccagcaaaaggccaggaaccgtaaaaaggccgcgttgctggcgtttttccataggctccgcccccctgacgagcatcacaaaaatcgacgctcaagtcagaggtggcgaaacccgacaggactataaagataccaggcgtttccccctggaagctccctcgtgcgctctcctgttccgaccctgccgcttaccggatacctgtccgcctttctcccttcgggaagcgtggcgctttctcatagctcacgctgtaggtatctcagttcggtgtaggtcgttcgctccaagctgggctgtgtgcacgaaccccccgttcagcccgaccgctgcgccttatccggtaactatcgtcttgagtccaacccggtaagacacgacttatcgccactggcagcagccactggtaacaggattagcagagcgaggtatgtaggcggtgctacagagttcttgaagtggtggcctaactacggctacactagaaggacagtatttggtatctgcgctctgctgaagccagttaccttcggaaaaagagttggtagctcttgatccggcaaacaaaccaccgctggtagcggtggtttttttgtttgcaagcagcagattacgcgcagaaaaaaaggatctcaagaagatcctttgatcttttctacggggtctgacgctcagtggaacgaaaactcacgttaagggattttggtcatgagattatcaaaaaggatcttcacctagatccttttaa

SEQ ID NO: 57 - DNA, 4900 bp, synthetic construct
  source 1..4900: mol_type = other DNA
attaaaaatgaagttttaaatcaatctaaagtatatatgagtaaacttggtctgacagttaccaatgcttaatcagtgaggcacctatctcagcgatctgtctatttcgttcatccatagttgcctgactccccgtcgtgtagataactacgatacgggagggcttaccatctggccccagtgctgcaatgataccgcgagacccacgctcaccggctccagatttatcagcaataaaccagccagccggaagggccgagcgcagaagtggtcctgcaactttatccgcctccatccagtctattaattgttgccgggaagctagagtaagtagttcgccagttaatagtttgcgcaacgttgttgccattgctacaggcatcgtggtgtcacgctcgtcgtttggtatggcttcattcagctccggttcccaacgatcaaggcgagttacatgatcccccatgttgtgcaaaaaagcggttagctccttcggtcctccgatcgttgtcagaagtaagttggccgcagtgttatcactcatggttatggcagcactgcataattctcttactgtcatgccatccgtaagatgcttttctgtgactggtgagtactcaaccaagtcattctgagaatagtgtatgcggcgaccgagttgctcttgcccggcgtcaatacgggataataccgcgccacatagcagaactttaaaagtgctcatcattggaaaacgttcttcggggcgaaaactctcaaggatcttaccgctgttgagatccagttcgatgtaacccactcgtgcacccaactgatcttcagcatcttttactttcaccagcgtttctgggtgagcaaaaacaggaaggcaaaatgccgcaaaaaagggaataagggcgacacggaaatgttgaatactcatactcttcctttttcaatattattgaagcatttatcagggttattgtctcatgagcggatacatatttgaatgtatttagaaaaataaacaaataggggttccgcgcacatttccccgaaaagtgccacctgacgcgccctgtagcggcgcattaagcgcggcgggtgtggtggttacgcgcagcgtgaccgctacacttgccagcgccctagcgcccgctcctttcgctttcttcccttcctttctcgccacgttcgccggctttccccgtcaagctctaaatcgggggctccctttagggttccgatttagtgctttacggcacctcgaccccaaaaaacttgattagggtgatggttcacgtagtgggccatcgccctgatagacggtttttcgccctttgacgttggagtccacgttctttaatagtggactcttgttccaaactggaacaacactcaaccctatctcggtctattcttttgatttataagggattttgccgatttcggcctattggttaaaaaatgagctgatttaacaaaaatttaacgcgaattttaacaaaatattaacgcttacaatttccattcgccattcaggctgcgcaactgttgggaagggcgatcggtgcgggcctcttcgctattacgccagctggcgaaagggggatgtgctgcaaggcgattaagttgggtaacgccagggttttcccagtcacgacgttgtaaaacgacggccagtgagcgcgcgtaatacgactcactatagggcgaattgggtaccgggccccccctcgaggtcgacggtatcgataagcttgatatcgaattgcattcattttatgtttcaggttcagggggaggtgtgggaggttttttaaagcaagtaaaacctctacaaatgtggtacgcgttgacattgattattgactagttattaatagtaatcaattacggggtcattagttcatagcccatatatggagttccgcgttacataacttacggtaaatggcccgcctggctgaccgcccaacgacccccgcccattgacgtcaataatgacgtatgttcccatagtaacgccaatagggactttccattgacgtcaatgggtggagtatttacggtaaactgcccacttggcagtacatcaagtgtatcatatgccaagtacgccccctattgacgtcaatgacggtaaatggcccgcctggcattatgcccagtacatgaccttatgggactttcctacttggcagtacatctacgtattagtcatcgctattaccatggtgatgcggttttggcagtacatcaatgggcgtggatagcggtttgactcacggggatttccaagtctccaccccattgacgtcaatgggagtttgttttggcaccaaaatcaacgggactttccaaaatgtcgtaacaactccgccccattgacgcaaatgggcggtaggcgtgtacggtgggaggtctatataagcagagctctctggctaactagagaacccactgcgccaccatgaccgagtacaagcccacggtgcgcctcgccacccgcgacgacgtccccagggccgtacgcaccctcgccgccgcgttcgccgactaccccgccacgcgccacaccgtcgatccggaccgccacatcgagcgggtcaccgagctgcaagaactcttcctcacgcgcgtcgggctcgacatcggcaaggtgtgggtcgcggacgacggcgccgcggtggcggtctggaccacgccggagagcgtcgaagcgggggcggtgttcgccgagatcggcccgcgcatggccgagttgagcggttcccggctggccgcgcagcaacagatggaaggcctcctggcgccgcaccggcccaaggagcccgcgtggttcctggccaccgtcggcgtctcgcccgaccaccagggcaagggtctgtaggtgcttcgatatcgatcgtttgggtggcaaaagctgataagctggctgaagagcattcatcgtggggatccgactataaggaccacgacggagactacaaggatcatgatattgattacaaagacgatgacgataagtaagaggggtctttgtcctctgtactgtctctctccttgccccccaaacgatcgatatcgaagcactaatggaccacgccggagagcgtcgaagcgggggcggtgttcgccgagatcggcccgcgcatggccgagttgagcggttcccggctggccgcgcagcaacagatggaaggcctcctggcgccgcaccggcccaaggagcccgcgtggttcctggccaccgtcggcgtctcgcccgaccaccagggcaagggtctgggcagcgccgtcgtgctccccggagtggaggcggccgagcgcgccggggtgcccgccttcctggagacctccgcgccccgcaacctccccttctacgagcggctcggcttcaccgtcaccgccgacgtcgaggtgcccgaaggaccgcgcacctggtgcatgacccgcaagcccggtgcctgaactcgagtctagagggcccgtttaaacccgctgatcagcctcgactgtgccttctagttgccagccatctgttgtttgcccctcccccgtgccttccttgaccctggaaggtgccactcccactgtcctttcctaataaaatgaggaaattgcatcgcattgtctgagtaggtgtcattctattctggggggtggggtggggcaggacagcaagggggaggattgggaagacaatagcaggcatgctggggatgcggtgggctctatgggcggccgccaccgcggtggagctccagcttttgttccctttagtgagggttaattgcgcgcttggcgtaatcatggtcatagctgtttcctgtgtgaaattgttatccgctcacaattccacacaacatacgagccggaagcataaagtgtaaagcctggggtgcctaatgagtgagctaactcacattaattgcgttgcgctcactgcccgctttccagtcgggaaacctgtcgtgccagctgcattaatgaatcggccaacgcgcggggagaggcggtttgcgtattgggcgctcttccgcttcctcgctcactgactcgctgcgctcggtcgttcggctgcggcgagcggtatcagctcactcaaaggcggtaatacggttatccacagaatcaggggataacgcaggaaagaacatgtgagcaaaaggccagcaaaaggccaggaaccgtaaaaaggccgcgttgctggcgtttttccataggctccgcccccctgacgagcatcacaaaaatcgacgctcaagtcagaggtggcgaaacccgacaggactataaagataccaggcgtttccccctggaagctccctcgtgcgctctcctgttccgaccctgccgcttaccggatacctgtccgcctttctcccttcgggaagcgtggcgctttctcatagctcacgctgtaggtatctcagttcggtgtaggtcgttcgctccaagctgggctgtgtgcacgaaccccccgttcagcccgaccgctgcgccttatccggtaactatcgtcttgagtccaacccggtaagacacgacttatcgccactggcagcagccactggtaacaggattagcagagcgaggtatgtaggcggtgctacagagttcttgaagtggtggcctaactacggctacactagaaggacagtatttggtatctgcgctctgctgaagccagttaccttcggaaaaagagttggtagctcttgatccggcaaacaaaccaccgctggtagcggtggtttttttgtttgcaagcagcagattacgcgcagaaaaaaaggatctcaagaagatcctttgatcttttctacggggtctgacgctcagtggaacgaaaactcacgttaagggattttggtcatgagattatcaaaaaggatcttcacctagatccttttaa